European Patent Specification EP 3 401 395 B1, published January 17, 2024. Title: HERBICIDE-TOLERANT PLANTS. Applicant: BASF AGROCHEMICAL PRODUCTS, B.V. The sequence listing filed with the application follows.

SEQUENCE LISTING (26 sequences)

SEQ ID NO: 1 - protein, 2320 aa, Alopecurus myosuroides
MGSTHLPIVGFNASTTPSLSTLRQINSAAAAFQSSSPSRSSKKKSRRVKSIRDDGDGSVPDPAGHGQSIRQGLAGIIDLPKEGASAPDVDISHGSEDHKASYQMNGILNESHNGRHASLSKVYEFCTELGGKTPIHSVLVANNGMAAAKFMRSVRTWANDTFGSEKAIQLIAMATPEDMRINAEHIRIADQFVEVPGGTNNNNYANVQLIVEIAERTGVSAVWPGWGHASENPELPDALTAKGIVFLGPPASSMNALGDKVGSALIAQAAGVPTLAWSGSHVEIPLELCLDSIPEEMYRKACVTTADEAVASCQMIGYPAMIKASWGGGGKGIRKVNNDDEVKALFKQVQGEVPGSPIFIMRLASQSRHLEVQLLCDEYGNVAALHSRDCSVQRRHQKIIEEGPVTVAPRETVKELEQAARRLAKAVGYVGAATVEYLYSMETGEYYFLELNPRLQVEHPVTESIAEVNLPAAQVAVGMGIPLWQIPEIRRFYGMDNGGGYDIWRKTAALATPFNFDEVDSQWPKGHCVAVRITSENPDDGFKPTGGKVKEISFKSKPNVWGYFSVKSGGGIHEFADSQFGHVFAYGETRSAAITSMSLALKEIQIRGEIHTNVDYTVDLLNAPDFRENTIHTGWLDTRIAMRVQAERPPWYISVVGGALYKTITTNAETVSEYVSYLIKGQIPPKHISLVHSTISLNIEESKYTIEIVRSGQGSYRLRLNGSLIEANVQTLCDGGLLMQLDGNSHVIYAEEEAGGTRLLIDGKTCLLQNDHDPSRLLAETPCKLLRFLIADGAHVDADVPYAEVEVMKMCMPLLSPAAGVINVLLSEGQAMQAGDLIARLDLDDPSAVKRAEPFEGSFPEMSLPIAASGQVHKRCAASLNAARMVLAGYDHAANKVVQDLVWCLDTPALPFLQWEELMSVLATRLPRRLKSELEGKYNEYKLNVDHVKIKDFPTEMLRETIEENLACVSEKEMVTIERLVDPLMSLLKSYEGGRESHAHFIVKSLFEEYLSVEELFSDGIQSDVIERLRLQYSKDLQKVVDIVLSHQGVRNKTKLILALMEKLVYPNPAAYRDQLIRFSSLNHKRYYKLALKASELLEQTKLSELRTSIARNLSALDMFTEEKADFSLQDRKLAINESMGDLVTAPLPVEDALVSLFDCTDQTLQQRVIQTYISRLYQPQLVKDSIQLKYQDSGVIALWEFTEGNHEKRLGAMVILKSLESVSTAIGAALKDASHYASSAGNTVHIALLDADTQLNTTEDSGDNDQAQDKMDKLSFVLKQDVVMADLRAADVKVVSCIVQRDGAIMPMRRTFLLSEEKLCYEEEPILRHVEPPLSALLELDKLKVKGYNEMKYTPSRDRQWHIYTLRNTENPKMLHRVFFRTLVRQPSAGNRFTSDHITDVEVGHAEEPLSFTSSSILKSLKIAKEELELHAIRTGHSHMYLCILKEQKLLDLVPVSGNTVVDVGQDEATACSLLKEMALKIHELVGARMHHLSVCQWEVKLKLVSDGPASGSWRVVTTNVTGHTCTVDIYREVEDTESQKLVYHSTALSSGPLHGVALNTSYQPLSVIDLKRCSARNNKTTYCYDFPLTFEAAVQKSWSNISSENNQCYVKATELVFAEKNGSWGTPIIPMQRAAGLNDIGMVAWILDMSTPEFPSGRQIIVIANDITFRAGSFGPREDAFFEAVTNLACEKKLPLIYLAANSGARIGIADEVKSCFRVGWTDDSSPERGFRYIYMTDEDHDRIGSSVIAHKMQLDSGEIRWVIDSVVGKEDGLGVENIHGSAAIASAYSRAYEETFTLTFVTGRTVGIGAYLARLGIRCIQRIDQPIILTGFSALNKLLGREVYSSHMQLGGPKIMATNGVVHLTVPDDLEGVSNILRWLSYVPANIGGPLPITKSLDPIDRPVAYIPENTCDPRAAISGIDDSQGKWLGGMFDKDSFVETFEGWAKTVVTGRAKLGGIPVGVIAVETQTMMQLVPADPGQPDSHERSVPRAGQVWFPDSATKTAQAMLDFNREGLPLFILANWRGFSGGQRDLFEGILQAGSTIVENLRTYNQPAFVYIPKAAELRGGAWVVIDSKINPDRIECYAERTAKGNVLEPQGLIEIKFRSEELKECMGRLDPELIDLKARLQGANGSLSDGESLQKSIEARKKQLLPLYTQIAVRFAELHDTSLRMAAKGVIRKVVDWEDSRSFFYKRLRRRLSEDVLAKEIRGVIGEKFPHKSAIELIKKWYLASEAAAAGSTDWDDDDAFVAWRENPENYKEYIKELRAQRVSRLLSDVAGSSSDLQALPQGLSMLLDKMDPSKRAQFIEEVMKVLK

SEQ ID NO: 2 - protein, 2327 aa, Oryza sativa
MTSTHVATLGVGAQAPPRHQKKSAGTAFVSSGSSRPSYRKNGQRTRSLREESNGGVSDSKKLNHSIRQGLAGIIDLPNDAASEVDISHGSEDPRGPTVPGSYQMNGIINETHNGRHASVSKVVEFCTALGGKTPIHSVLVANNGMAAAKFMRSVRTWANDTFGSEKAIQLIAMATPEDLRINAEHIRIADQFVEVPGGTNNNNYANVQLIVEIAERTGVSAVWPGWGHASENPELPDALTAKGIVFLGPPASSMHALGDKVGSALIAQAAGVPTLAWSGSHVEVPLECCLDSIPDEMYRKACVTTTEEAVASCQVVGYPAMIKASWGGGGKGIRKVHNDDEVRTLFKQVQGEVPGSPIFIMRLAAQSRHLEVQLLCDQYGNVAALHSRDCSVQRRHQKIIEEGPVTVAPRETVKELEQAARRLAKAVGYVGAATVEYLYSMETGEYYFLELNPRLQVEHPVTEWIAEVNLPAAQVAVGMGIPLWQIPEIRRFYGMNHGGGYDLWRKTAALATPFNFDEVDSKWPKGHCVAVRITSEDPDDGFKPTGGKVKEISFKSKPNVWAYFSVKSGGGIHEFADSQFGHVFAYGTTRSAAITTMALALKEVQIRGEIHSNVDYTVDLLNASDFRENKIHTGWLDTRIAMRVQAERPPWYISVVGGALYKTVTANTATVSDYVGYLTKGQIPPKHISLVYTTVALNIDGKKYTIDTVRSGHGSYRLRMNGSTVDANVQILCDGGLLMQLDGNSHVIYAEEEASGTRLLIDGKTCMLQNDHDPSKLLAETPCKLLRFLVADGAHVDADVPYAEVEVMKMCMPLLSPASGVIHVVMSEGQAMQAGDLIARLDLDDPSAVKRAEPFEDTFPQMGLPIAASGQVHKLCAASLNACRMILAGYEHDIDKVVPELVYCLDTPELPFLQWEELMSVLATRLPRNLKSELEGKYEEYKVKFDSGIINDFPANMLRVIIEENLACGSEKEKATNERLVEPLMSLLKSYEGGRESHAHFVVKSLFEEYLYVEELFSDGIQSDVIERLRLQHSKDLQKVVDIVLSHQSVRNKTKLILKLMESLVYPNPAAYRDQLIRFSSLNHKAYYKLALKASELLEQTKLSELRARIARSLSELEMFTEESKGLSMHKREIAIKESMEDLVTAPLPVEDALISLFDCSDTTVQQRVIETYIARLYQPHLVKDSIKMKWIESGVIALWEFPEGHFDARNGGAVLGDKRWGAMVIVKSLESLSMAIRFALKETSHYTSSEGNMMHIALLGADNKMHIIQESGDDADRIAKLPLILKDNVTDLHASGVKTISFIVQRDEARMTMRRTFLWSDEKLSYEEEPILRHVEPPLSALLELDKLKVKGYNEMKYTPSRDRQWHIYTLRNTENPKMLHRVFFRTLVRQPSVSNKFSSGQIGDMEVGSAEEPLSFTSTSILRSLMTAIEELELHAIRTGHSHMYLHVLKEQKLLDLVPVSGNTVLDVGQDEATAYSLLKEMAMKIHELVGARMHHLSVCQWEVKLKLDCDGPASGTWRIVTTNVTSHTCTVDIYREMEDKESRKLVYHPATPAAGPLHGVALNNPYQPLSVIDLKRCSARNNRTTYCYDFPLAFETAVRKSWSSSTSGASKGVENAQCYVKATELVFADKHGSWGTPLVQMDRPAGLNDIGMVAWTLKMSTPEFPSGREIIVVANDITFRAGSFGPREDAFFEAVTNLACEKKLPLIYLAANSGARIGIADEVKSCFRVGWSDDGSPERGFQYIYLSEEDYARIGTSVIAHKMQLDSGEIRWVIDSVVGKEDGLGVENIHGSAAIASAYSRAYKETFTLTFVTGRTVGIGAYLARLGIRCIQRLDQPIILTGYSALNKLLGREVYSSHMQLGGPKIMATNGVVHLTVSDDLEGVSNILRWLSYVPAYIGGPLPVTTPLDPPDRPVAYIPENSCDPRAAIRGVDDSQGKWLGGMFDKDSFVETFEGWAKTVVTGRAKLGGIPVGVIAVETQTMMQTIPADPGQLDSREQSVPRAGQVWFPDSATKTAQALLDFNREGLPLFILANWRGFSGGQRDLFEGILQAGSTIVENLRTYNQPAFVYIPMAAELRGGAWVVVDSKINPDRIECYAERTAKGNVLEPQGLIEIKFRSEELQDCMSRLDPTLIDLKAKLEVANKNGSADTKSLQENIEARTKQLMPLYTQIAIRFAELHDTSLRMAAKGVIKKVVDWEESRSFFYKRLRRRISEDVLAKEIRAVAGEQFSHQPAIELIKKWYSASHAAEWDDDDAFVAWMDNPENYKDYIQYLKAQRVSQSLSSLSDSSSDLQALPQGLSMLLDKMDPSRRAQLVEEIRKVLG

SEQ ID NO: 3 - protein, 2327 aa, Oryza sativa; identical to SEQ ID NO: 2

SEQ ID NO: 4 - DNA, 6963 bp, Alopecurus myosuroides
atgggatccacacatctgcccattgtcgggtttaatgcatccacaacaccatcgctatccactcttcgccagataaactcagctgctgctgcattccaatcttcgtccccttcaaggtcatccaagaagaaaagccgacgtgttaagtcaataagggatgatggcgatggaagcgtgccagaccctgcaggccatggccagtctattcgccaaggtctcgctggcatcatcgacctcccaaaggagggcgcatcagctccagatgtggacatttcacatgggtctgaagaccacaaggcctcctaccaaatgaatgggatactgaatgaatcacataacgggaggcacgcctctctgtctaaagtttatgaattttgcacggaattgggtggaaaaacaccaattcacagtgtattagtcgccaacaatggaatggcagcagctaagttcatgcggagtgtccggacatgggctaatgatacatttgggtcagagaaggcgattcagttgatagctatggcaactccggaagacatgagaataaatgcagagcacattagaattgctgatcagtttgttgaagtacctggtggaacaaacaataacaactatgcaaatgtccaactcatagtggagatagcagagagaactggtgtctccgccgtttggcctggttggggccatgcatctgagaatcctgaacttccagatgcactaactgcaaaaggaattgtttttcttgggccaccagcatcatcaatgaacgcactaggcgacaaggttggttcagctctcattgctcaagcagcaggggttcccactcttgcttggagtggatcacatgtggaaattccattagaactttgtttggactcgatacctgaggagatgtataggaaagcctgtgttacaaccgctgatgaagcagttgcaagttgtcagatgattggttaccctgccatgatcaaggcatcctggggtggtggtggtaaagggattagaaaggttaataatgatgacgaggtgaaagcactgtttaagcaagtacagggtgaagttcctggctccccgatatttatcatgagacttgcatctcagagtcgtcatcttgaagtccagctgctttgtgatgaatatggcaatgtagcagcacttcacagtcgtgattgcagtgtgcaacgacgacaccaaaagattatcgaggaaggaccagttactgttgctcctcgtgaaacagtgaaagagctagagcaagcagcaaggaggcttgctaaggccgtgggttacgtcggtgctgctactgttgaatatctctacagcatggagactggtgaatactattttctggagcttaatccacggttgcaggttgagcacccagtcaccgagtcgatagctgaagtaaatttgcctgcagcccaagttgcagttgggatgggtatacccctttggcagattccagagatcagacgtttctacggaatggacaatggaggaggctatgatatttggaggaaaacagcagctctcgctactccattcaactttgatgaagtagattctcaatggccgaagggtcattgtgtggcagttaggataaccagtgagaatccagatgatggattcaagcctactggtggaaaagtaaaggagataagttttaaaagtaagccaaatgtctggggatatttctcagttaagtctggtggaggcattcatgaatttgcggattctcagtttggacacgtttttgcctatggagagactagatcagcagcaataaccagcatgtctcttgcactaaaagagattcaaattcgtggagaaattcatacaaacgttgattacacggttgatctcttgaatgccccagacttcagagaaaacacgatccataccggttggctggataccagaatagctatgcgtgttcaagctgagaggcctccctggtatatttcagtggttggaggagctctatataaaacaataaccaccaatgcggagaccgtttctgaatatgttagctatctcatcaagggtcagattccaccaaagcacatatcccttgtccattcaactatttctttgaatatagaggaaagcaaatatacaattgagattgtgaggagtggacagggtagctacagattgagactgaatggatcacttattgaagccaatgtacaaacattatgtgatggaggccttttaatgcagctggatggaaatagccatgttatttatgctgaagaagaagcgggtggtacacggcttcttattgatggaaaaacatgcttgctacagaatgaccatgatccgtcaaggttattagctgagacaccctgcaaacttcttcgtttcttgattgccgatggtgctcatgttgatgctgatgtaccatacgcggaagttgaggttatgaagatgtgcatgcccctcttgtcgcctgctgctggtgtcattaatgttttgttgtctgagggccaggcgatgcaggctggtgatcttatagcgagacttgatctcgatgacccttctgctgtgaagagagccgagccatttgaaggatcttttccagaaatgagccttcctattgctgcttctggccaagttcacaaaagatgtgctgcaagtttgaacgctgctcgaatggtccttgcaggatatgaccatgcggccaacaaagttgtgcaagatttggtatggtgccttgatacacctgctcttcctttcctacaatgggaagagcttatgtctgttttagcaactagacttccaagacgtcttaagagcgagttggagggcaaatacaatgaatacaagttaaatgttgaccatgtgaagatcaaggatttccctaccgagatgcttagagagacaatcgaggaaaatcttgcatgtgtttccgagaaggaaatggtgacaattgagaggcttgttgaccctctgatgagcctgctgaagtcatacgagggtgggagagaaagccatgcccactttattgtcaagtccctttttgaggagtatctctcggttgaggaactattcagtgatggcattcagtctgacgtgattgaacgcctgcgcctacaatatagtaaagacctccagaaggttgtagacattgttttgtctcaccagggtgtgagaaacaaaacaaagctgatactcgcgctcatggagaaactggtctatccaaaccctgctgcctacagagatcagttgattcgcttttcttccctcaaccataaaagatattataagttggctcttaaagctagtgaacttcttgaacaaaccaagctcagcgaactccgcacaagcattgcaaggaacctttcagcgctggatatgttcaccgaggaaaaggcagatttctccttgcaagacagaaaattggccattaatgagagcatgggagatttagtcactgccccactgccagttgaagatgcacttgtttctttgtttgattgtactgatcaaactcttcagcagagagtgattcagacatacatatctcgattataccagcctcaacttgtgaaggatagcatccagctgaaatatcaggattctggtgttattgctttatgggaattcactgaaggaaatcatgagaagagattgggtgctatggttatcctgaagtcactagaatctgtgtcaacagccattggagctgctctaaaggatgcatcacattatgcaagctctgcgggcaacacggtgcatattgctttgttggatgctgatacccaactgaatacaactgaagatagtggtgataatgaccaagctcaagacaagatggataaactttcttttgtactgaaacaagatgttgtcatggctgatctacgtgctgctgatgtcaaggttgttagttgcattgttcaaagagatggagcaatcatgcctatgcgccgtaccttcctcttgtcagaggaaaaactttgttacgaggaagagccgattcttcggcatgtggagcctccactttctgcacttcttgagttggataaattgaaagtgaaaggatacaatgagatgaagtatacaccgtcacgtgatcgtcagtggcatatatacacacttagaaatactgaaaatccaaaaatgctgcacagggtatttttccgaacacttgtcagacaacccagtgcaggcaacaggtttacatcagaccatatcactgatgttgaagtaggacacgcagaggaacctctttcatttacttcaagcagcatattaaaatcgttgaagattgctaaagaagaattggagcttcacgcgatcaggactggccattctcatatgtacttgtgcatattgaaagagcaaaagcttcttgaccttgttcctgtttcagggaacactgttgtggatgttggtcaagatgaagctactgcatgctctcttttgaaagaaatggctttaaagatacatgaacttgttggtgcaagaatgcatcatctttctgtatgccagtgggaagtgaaacttaagttggtgagcgatgggcctgccagtggtagctggagagttgtaacaaccaatgttactggtcacacctgcactgtggatatctaccgggaggtcgaagatacagaatcacagaaactagtataccactccaccgcattgtcatctggtcctttgcatggtgttgcactgaatacttcgtatcagcctttgagtgttattgatttaaaacgttgctctgccaggaacaacaaaactacatactgctatgattttccattgacatttgaagctgcagtgcagaagtcgtggtctaacatttccagtgaaaacaaccaatgttatgttaaagcgacagagcttgtgtttgctgaaaagaatgggtcgtggggcactcctataattcctatgcagcgtgctgctgggctgaatgacattggtatggtagcctggatcttggacatgtccactcctgaatttcccagcggcagacagatcattgttatcgcaaatgatattacatttagagctggatcatttggcccaagggaagatgcatttttcgaagctgtaaccaacctggcttgtgagaagaagcttccacttatctacttggctgcaaactctggtgctcggattggcattgctgatgaagtaaaatcttgcttccgtgttggatggactgatgatagcagccctgaacgtggatttaggtacatttatatgactgacgaagaccatgatcgtattggctcttcagttatagcacacaagatgcagctagatagtggcgagatcaggtgggttattgattctgttgtgggaaaagaggatggactaggtgtggagaacatacatggaagtgctgctattgccagtgcctattctagggcgtacgaggagacatttacacttacattcgttactggacgaactgttggaatcggagcctatcttgctcgacttggcatacggtgcatacagcgtattgaccagcccattattttgaccgggttttctgccctgaacaagcttcttgggcgggaggtgtacagctcccacatgcagttgggtggtcccaaaatcatggcgacgaatggtgttgtccatctgactgttccagatgaccttgaaggtgtttctaatatattgaggtggctcagctatgttcctgcaaacattggtggacctcttcctattacaaaatctttggacccaatagacagacccgttgcatacatccctgagaatacatgtgatcctcgtgcagccatcagtggcattgatgacagccaagggaaatggttgggtggcatgtttgacaaagacagttttgtggagacatttgaaggatgggcgaagacagtagttactggcagagcaaaacttggagggattcctgttggtgttatagctgtggagacacagaccatgatgcagctcgtccccgctgatccaggccagcctgattcccacgagcggtctgttcctcgtgctgggcaagtttggtttccagattctgctaccaagacagcgcaggcgatgttggacttcaaccgtgaaggattacctctgttcatacttgctaactggagaggcttctctggagggcaaagagatctttttgaaggaattctgcaggctgggtcaacaattgttgagaaccttaggacatacaatcagcctgcctttgtatatatccccaaggctgcagagctacgtggaggagcctgggtcgtgattgatagcaagataaacccagatcgcatcgagtgctatgctgagaggactgcaaagggtaatgttctcgaacctcaagggttgattgagatcaagttcaggtcagaggaactcaaagaatgcatgggtaggcttgatccagaattgatagatctgaaagcaagactccagggagcaaatggaagcctatctgatggagaatcccttcagaagagcatagaagctcggaagaaacagttgctgcctctgtacacccaaatcgcggtacgttttgcggaattgcacgacacttcccttagaatggctgctaaaggtgtgatcaggaaagttgtagactgggaagactctcggtctttcttctacaagagattacggaggaggctatccgaggacgttctggcaaaggagattagaggtgtaattggtgagaagtttcctcacaaatcagcgatcgagctgatcaagaaatggtacttggcttctgaggcagctgcagcaggaagcaccgactgggatgacgacgatgcttttgtcgcctggagggagaaccctgaaaactataaggagtatatcaaagagcttagggctcaaagggtatctcggttgctctcagatgttgcaggctccagttcggatttacaagccttgccgcagggtctttccatgctactagataagatggatccctctaagagagcacagtttatcgaggaggtcatgaaggtcctgaaatga

SEQ ID NO: 5 - DNA, 11927 bp, Oryza sativa
atgacatccacacatgtggcgacattgggagttggtgcccaggcacctcctcgtcaccagaaaaagtcagctggcactgcatttgtatcatctgggtcatcaagaccctcataccgaaagaatggtcagcgtactcggtcacttagggaagaaagcaatggaggagtgtctgattccaaaaagcttaaccactctattcgccaaggtgaccactagctactttacatatgctataatttgtgccaaacataaacatgcaatggctgctattatttaaacgttaatgttgaaatagctgctataggatacagcaaaaatatataattgactgggcaagatgcaacaattgtttttcactaaagttagttatcttttgctgtaaaagacaactgttttttacataaaatggtattaataaccttgtaatattcaatgcaacatgttctcaagtaaaaaaaaacattgcctggttgtataagcaaatgtgtcgttgtagacatcttattaaacctttttgtgatatctattaccgtagggaacaggggagctgtttaaatctgttatcatagagtaatatgagaaaagtggattgtgcgactttggcatgtatacctgctcaatttcaaatatatgtctatgtgcaggtcttgctggcatcattgacctcccaaatgacgcagcttcagaagttgatatttcacagtaaggactttatattttataataattattatataattttctgacatgttttgagaacctcaaaacatgtgattgcaccttccttttttatgtctggttcagaaactgataagttttgacagtgtttaggatggatctttgatgcgcacagtgctttctaatgttttcatttttgaaagtaatgttttaggaagaaatatctgattaaatttatactttatctttacaaaagtcaaatgcgttctgtatcaattgcggtttgtaatatggcaagaacatgctttcagaatttgttcatacaatgctttctttctattattatgtagaacaaatacctaatactttgttcaccttttatagtggacacctctcacagctttttcagtaagtgatgcaattttgtacatttgtaagatgtgttccagaaaccttttctcctgcaattctaatgtacccactcaaactggtatcaccaaagatctccatctgattgaaaaaaagctgcgtgaagtatgcttatttatgctaaccatacatgatttatactgttttatagtacaatgcttatttatgctaaccatacataattttattctgttttctagtacattatttgtgcccctgaccataaatgatcctttcttttacagtggttccgaagatcccagggggcctacggtcccaggttcctaccaaatgaatgggattatcaatgaaacacataatgggaggcatgcttcagtctccaaggttgttgagttttgtacggcacttggtggcaaaacaccaattcacagtgtattagtggccaacaatggaatggcagcagctaagttcatgcggagtgtccgaacatgggctaatgatacttttggatcagagaaggcaattcagctgatagctatggcaactccggaggatctgaggataaatgcagagcacatcagaattgccgatcaatttgtagaggtacctggtggaacaaacaacaacaactatgcaaatgtccaactcatagtggaggttagttcagctcatccctcaacacaacattttcgtttctatttaagttagggaaaaatctctacgaccctccaatttctgaacatccaattttcaccatcaactgcaatcacagatagcagagagaacaggtgtttctgctgtttggcctggttggggtcatgcatctgagaatcctgaacttccagatgcgctgactgcaaaaggaattgtttttcttgggccaccagcatcatcaatgcatgcattaggagacaaggttggctcagctctcattgctcaagcagctggagttccaacacttgcttggagtggatcacatgtgagccttgtcttctcttttttagcttatcatcttatcttttcggtgatgcattatcccaatgacactaaaccataggtggaagttcctctggagtgttgcttggactcaatacctgatgagatgtatagaaaagcttgtgttactaccacagaggaagcagttgcaagttgtcaggtggttggttatcctgccatgattaaggcatcttggggtggtggtggtaaaggaataaggaaggtttgttcttcttgtagttatcaagagattgtttggattgcaagtgtttagtgcccatagttaactctggtctttctaacatgagtaactcaactttcttgcaggttcataatgatgatgaggttaggacattatttaagcaagttcaaggcgaagtacctggttccccaatatttatcatgaggctagctgctcaggtggggccttttatggaagttacaccttttcccttaatgttgagttattccggagttattatggttatgttctgtatgtttgatctgtaaattattgaaattcacctccattggttctccagattagcagacctacaattctacatatggtttatactttataaatactaggatttagggatcttcatatagtttatacatggtatttagatttcatttgtaaccctattgaagacatcctgattgttgtcttatgtagagtcgacatcttgaagttcagttgctttgtgatcaatatggcaacgtagcagcacttcacagtcgagattgcagtgtacaacggcgacaccaaaaggtctgctgtctcagttaaatcacccctctgaatgatctacttcttgcctgctgcgttggtcagaggaataatggttgtattctactgaacagataatcgaggaaggaccagttactgttgctcctcgtgagactgtgaaagagcttgagcaggcagcacggaggcttgctaaagctgtgggttatgttggtgctgctactgttgaatacctttacagcatggaaactggtgaatattattttctggaacttaatccacggctacaggtcggctcctttgacattcttcaggaattaatttctgttgaccacatgatttacattgtcaaatggtctcacaggttgagcatcctgtcactgagtggatagctgaagtaaatttgcctgcggctcaagttgctgttggaatgggtatacccctttggcagattccaggtaatgcttcttcatttagttcctgctctttgttaattgaatgagctcttatacagaccatgagacacattctactgttaattcatagtatcccctgacttgttagtgttagagatacagagatgtatcacaaattcattgtatctcctcaaggactgtaaaaatcctataattaaatttctgaaaatttgttcttttaagcagaaaaaaaatctctaaattatctccctgtatacagagatcaggcgcttctacggaatgaaccatggaggaggctatgacctttggaggaaaacagcagctctagcgactccatttaactttgatgaagtagattctaaatggccaaaaggccactgcgtagctgttagaataactagcgaggatccagatgatgggtttaagcctactggtggaaaagtaaaggtgcggtttcctgatgttaggtgtatgaattgaacacattgctatattgcagctagtgaaatgactggatcatggttctcttattttcaggagataagtttcaagagtaaaccaaatgtttgggcctatttctcagtaaaggtagtcctcaatattgttgcactgccacattatttgagttgtcctaacaattgtgctgcaattgttagttttcaactatttgttgttctgtttggttgactggtaccctctctttgcagtctggtggaggcatccatgaattcgctgattctcagttcggtatgtaaagttaaaagagtaatattgtctttgctatttatgtttgtcctcacttttaaaagatattgccttccattacaggacatgtttttgcgtatggaactactagatcggcagcaataactaccatggctcttgcactaaaagaggttcaaattcgtggagaaattcattcaaacgtagactacacagttgacctattaaatgtaaggactaaatatctgcttattgaaccttgctttttggttccctaatgccattttagtctggctactgaagaacttatccatcatgccatttctgttatcttaaattcaggcctcagattttagagaaaataagattcatactggttggctggataccaggatagccatgcgtgttcaagctgagaggcctccatggtatatttcagtcgttggaggggctttatatgtaagacaaactatgccactcattagcatttatgtgaagcaaatgcggaaaacatgatcaatatgtcgtcttatttaaatttatttatttttgtgctgcagaaaacagtaactgccaacacggccactgtttctgattatgttggttatcttaccaagggccagattccaccaaaggtactattctgttttttcaggatatgaatgctgtttgaatgtgaaaaccattgaccataaatccttgtttgcagcatatatcccttgtctatacgactgttgctttgaatatagatgggaaaaaatatacagtaagtgtgacattcttaatggggaaacttaatttgttgtaaataatcaatatcatattgactcgtgtatgctgcatcatagatcgatactgtgaggagtggacatggtagctacagattgcgaatgaatggatcaacggttgacgcaaatgtacaaatattatgtgatggtgggcttttaatgcaggtaatatcttcttcctagttaaagaagatatatcttgttcaaagaattctgattattgatcttttaatgttttcagctggatggaaacagccatgtaatttatgctgaagaagaggccagtggtacacgacttcttattgatggaaagacatgcatgttacaggtaatgatagccttgttctttttagttctagtcacggtgtttgcttgctatttgttgtatctatttaatgcattcactaattactatattagtttgcatcatcaagttaaaatggaacttctttcttgcagaatgaccatgacccatcaaagttattagctgagacaccatgcaaacttcttcgtttcttggttgctgatggtgctcatgttgatgctgatgtaccatatgcggaagttgaggttatgaagatgtgcatgcccctcttatcacccgcttctggtgtcatacatgttgtaatgtctgagggccaagcaatgcaggtacattcctacattccattcattgtgctgtgctgacatgaacatttcaagtaaatacctgtaacttgtttattattctaggctggtgatcttatagctaggctggatcttgatgacccttctgctgttaagagagctgagccgttcgaagatacttttccacaaatgggtctccctattgctgcttctggccaagttcacaaattatgtgctgcaagtctgaatgcttgtcgaatgatccttgcggggtatgagcatgatattgacaaggtaaacatcatgtcctcttgttttttcttttgtttatcatgcattcttatgttcatcatgtcctctggcaaatctagattccgctgtcgtttcacacagatttttctcattctcataatggtgccaaacataaatatgctgctatattcatcaatgttttcactcgatttctaattttgcttttgagttttaaactttagtacaatccatatctaatctcctttggcaacagtgaatccattatatatatttttattaaactgctttctttttcaggttgtgccagagttggtatactgcctagacactccggagcttcctttcctgcagtgggaggagcttatgtctgttttagcaactagacttccaagaaatcttaaaagtgaggtatattatggttgacaagatagctagtctcatgctctaaggacttgtacatttcgccacataggttaattttccatatcaagttctaatgtacgatataaaagtagtactggcctaaaacagtattggtggttgactatctttgttgtgtaagatcaagtatttctttttcatgcttagtttgtcaatacttcacatttatcactgacttgtcgagctaaatgagattttatttgatttctgtgctccattatttttgtatatatatatatatatttaactatgactatatgttatgcctcaaacgtttcaaactctttcagttggagggcaaatatgaggaatacaaagtaaaatttgactctgggataatcaatgatttccctgccaatatgctacgagtgataattgaggtcagttattcaatttgttgtgataatcactgccttaactgttcgttcttttaacaagcggttttataggaaaatcttgcatgtggttctgagaaggagaaggctacaaatgagaggcttgttgagcctcttatgagcctactgaagtcatatgagggtgggagagaaagtcatgctcactttgttgtcaagtccctttttgaggagtatctctatgttgaagaattgttcagtgatggaattcaggttaacttacctattcgcattaaacaaatcatcagttgttttatgataaagtcaaaatgtttatatttcccattcttctgtggatcaaatatatcacggacatgatatagtttccttaggctatataatggttcttcatcaaataatattgcaggaaacagtatagcaaactatttgtatatactcgagatggaaattgttagaaacatcattgactaaatctgtcctttgttacgctgtttttgtagtctgatgtgattgagcgtctgcgccttcaacatagtaaagacctacagaaggtcgtagacattgtgttgtcccaccaggtaaatttcttcatggtctgatgacttcactgcgaatggttactgaactgtcttcttgttctgacaatgtgacttttctttgtagagtgttagaaataaaactaagctgatactaaaactcatggagagtctggtctatccaaatcctgctgcctacagggatcaattgattcgcttttcttcccttaatcacaaagcgtattacaaggtgaccaggataaacataaataaacgtgaatttttcaatgaccttttcttctgacatctgaatctgatgaatttcttgcatattaatacagttggcacttaaagctagtgaacttcttgaacaaacaaaacttagtgagctccgtgcaagaatagcaaggagcctttcagagctggagatgtttactgaggaaagcaagggtctctccatgcataagcgagaaattgccattaaggagagcatggaagatttagtcactgctccactgccagttgaagatgcgctcatttctttatttgattgtagtgatacaactgttcaacagagagtgattgagacttatatagctcgattataccaggtatgagaagaaagaccttttgaaattatttatattaacatatcctagtaaaacagcatgctcatcatttcttaaaaaaagtttacagcacctgatgtttggttactgaccgcatcattaaaataaagttacttgttgtggagagatgtattttggaacttgtggcacatgcagtaacatgctactgctcgatatgtttgctaacttgacaacaatatttttcagcctcatcttgtaaaggacagtatcaaaatgaaatggatagaatcgggtgttattgctttatgggaatttcctgaagggcattttgatgcaagaaatggaggagcggttcttggtgacaaaagatggggtgccatggtcattgtcaagtctcttgaatcactttcaatggccattagatttgcactaaaggagacatcacactacactagctctgagggcaatatgatgcatattgctttgttgggtgctgataataagatgcatataattcaagaaaggtatgttcatatgctatgttggtgctgaaatagttatatatgtagttagctggtggagttctggtaattaacctatcccattgttcagtggtgatgatgctgacagaatagccaaacttcccttgatactaaaggataatgtaaccgatctgcatgcctctggtgtgaaaacaataagtttcattgttcaaagagatgaagcacggatgacaatgcgtcgtaccttcctttggtctgatgaaaagctttcttatgaggaagagccaattctccggcatgtggaacctcctctttctgcacttcttgagttggtacgtgatatcatcaaaatgataatgttttggtatggcattgattatcttctatgctctttgtatttattcagcctattgtggatacaggacaagttgaaagtgaaaggatacaatgaaatgaagtataccccatcacgggatcgtcaatggcatatctacacacttagaaatactgaaaaccccaaaatgttgcaccgggtatttttccgaacccttgtcaggcaacccagtgtatccaacaagttttcttcgggccagattggtgacatggaagttgggagtgctgaagaacctctgtcatttacatcaaccagcatattaagatctttgatgactgctatagaggaattggagcttcacgcaattagaactggccattcacacatgtatttgcatgtattgaaagaacaaaagcttcttgatcttgttccagtttcagggtaagtgcgcatatttctttttgggaacatatgcttgcttatgaggttggtcttctcaatgatcttcttatcttactcaggaatacagttttggatgttggtcaagatgaagctactgcatattcacttttaaaagaaatggctatgaagatacatgaacttgttggtgcaagaatgcaccatctttctgtatgccaatgggaagtgaaacttaagttggactgcgatggtcctgccagtggtacctggaggattgtaacaaccaatgttactagtcacacttgcactgtggatgtaagtttaatcctctagcattttgttttctttggaaaagcatgtgattttaagccggctggtcctcatacccagacctagtgatctttatatagtgtagacatttttctaactgcttttaattgttttagatctaccgtgagatggaagataaagaatcacggaagttagtataccatcccgccactccggcggctggtcctctgcatggtgtggcactgaataatccatatcagcctttgagtgtcattgatctcaaacgctgttctgctaggaataatagaactacatactgctatgattttccactggtgagttgactgctcccttatattcaatgcattaccatagcaaattcatattcgttcatgttgtcaaaataagccgatgaaaattcaaaactgtaggcatttgaaactgcagtgaggaagtcatggtcctctagtacctctggtgcttctaaaggtgttgaaaatgcccaatgttatgttaaagctacagagttggtatttgcggacaaacatgggtcatggggcactcctttagttcaaatggaccggcctgctgggctcaatgacattggtatggtagcttggaccttgaagatgtccactcctgaatttcctagtggtagggagattattgttgttgcaaatgatattacgttcagagctggatcatttggcccaagggaagatgcattttttgaagctgttaccaacctagcctgtgagaagaaacttcctcttatttatttggcagcaaattctggtgctcgaattggcatagcagatgaagtgaaatcttgcttccgtgttgggtggtctgatgatggcagccctgaacgtgggtttcagtacatttatctaagcgaagaagactatgctcgtattggcacttctgtcatagcacataagatgcagctagacagtggtgaaattaggtgggttattgattctgttgtgggcaaggaagatggacttggtgtggagaatatacatggaagtgctgctattgccagtgcttattctagggcatataaggagacatttacacttacatttgtgactggaagaactgttggaataggagcttatcttgctcgacttggcatccggtgcatacagcgtcttgaccagcctattattcttacaggctattctgcactgaacaagcttcttgggcgggaagtgtacagctcccacatgcagttgggtggtcccaaaatcatggcaactaatggtgttgtccatcttactgtttcagatgaccttgaaggcgtttctaatatattgaggtggctcagttatgttcctgcctacattggtggaccacttccagtaacaacaccgttggacccaccggacagacctgttgcatacattcctgagaactcgtgtgatcctcgagcggctatccgtggtgttgatgacagccaagggaaatggttaggtggtatgtttgataaagacagctttgtggaaacatttgaaggttgggctaagacagtggttactggcagagcaaagcttggtggaattccagtgggtgtgatagctgtggagactcagaccatgatgcaaactatccctgctgaccctggtcagcttgattcccgtgagcaatctgttcctcgtgctggacaagtgtggtttccagattctgcaaccaagactgcgcaggcattgctggacttcaaccgtgaaggattacctctgttcatcctcgctaactggagaggcttctctggtggacaaagagatctttttgaaggaattcttcaggctggctcgactattgttgagaaccttaggacatacaatcagcctgcctttgtctacattcccatggctgcagagctacgaggaggggcttgggttgtggttgatagcaagataaacccagaccgcattgagtgctatgctgagaggactgcaaaaggcaatgttctggaaccgcaagggttaattgagatcaagttcaggtcagaggaactccaggattgcatgagtcggcttgacccaacattaattgatctgaaagcaaaactcgaagtagcaaataaaaatggaagtgctgacacaaaatcgcttcaagaaaatatagaagctcgaacaaaacagttgatgcctctatatactcagattgcgatacggtttgctgaattgcatgatacatccctcagaatggctgcgaaaggtgtgattaagaaagttgtggactgggaagaatcacgatctttcttctataagagattacggaggaggatctctgaggatgttcttgcaaaagaaattagagctgtagcaggtgagcagttttcccaccaaccagcaatcgagctgatcaagaaatggtattcagcttcacatgcagctgaatgggatgatgacgatgcttttgttgcttggatggataaccctgaaaactacaaggattatattcaatatcttaaggctcaaagagtatcccaatccctctcaagtctttcagattccagctcagatttgcaagccctgccacagggtctttccatgttactagataaggtaattagcttactgatgcttatataaattctttttcattacatatggctggagaactatctaatcaaataatgattataattccaatcgttctttttatgccattatgatcttctgaaatttccttctttggacacttattcagatggatccctctagaagagctcaacttgttgaagaaatcaggaaggtccttggttga

SEQ ID NO: 6 - DNA, 6984 bp, Oryza sativa
atgacatccacacatgtggcgacattgggagttggtgcccaggcacctcctcgtcaccagaaaaagtcagctggcactgcatttgtatcatctgggtcatcaagaccctcataccgaaagaatggtcagcgtactcggtcacttagggaagaaagcaatggaggagtgtctgattccaaaaagcttaaccactctattcgccaaggtcttgctggcatcattgacctcccaaatgacgcagcttcagaagttgatatttcacatggttccgaagatcccagggggcctacggtcccaggttcctaccaaatgaatgggattatcaatgaaacacataatgggaggcatgcttcagtctccaaggttgttgagttttgtacggcacttggtggcaaaacaccaattcacagtgtattagtggccaacaatggaatggcagcagctaagttcatgcggagtgtccgaacatgggctaatgatacttttggatcagagaaggcaattcagctgatagctatggcaactccggaggatctgaggataaatgcagagcacatcagaattgccgatcaatttgtagaggtacctggtggaacaaacaacaacaactatgcaaatgtccaactcatagtggagatagcagagagaacaggtgtttctgctgtttggcctggttggggtcatgcatctgagaatcctgaacttccagatgcgctgactgcaaaaggaattgtttttcttgggccaccagcatcatcaatgcatgcattaggagacaaggttggctcagctctcattgctcaagcagctggagttccaacacttgcttggagtggatcacatgtggaagttcctctggagtgttgcttggactcaatacctgatgagatgtatagaaaagcttgtgttactaccacagaggaagcagttgcaagttgtcaggtggttggttatcctgccatgattaaggcatcttggggtggtggtggtaaaggaataaggaaggttcataatgatgatgaggttaggacattatttaagcaagttcaaggcgaagtacctggttccccaatatttatcatgaggctagctgctcagagtcgacatcttgaagttcagttgctttgtgatcaatatggcaacgtagcagcacttcacagtcgagattgcagtgtacaacggcgacaccaaaagataatcgaggaaggaccagttactgttgctcctcgtgagactgtgaaagagcttgagcaggcagcacggaggcttgctaaagctgtgggttatgttggtgctgctactgttgaatacctttacagcatggaaactggtgaatattattttctggaacttaatccacggctacaggttgagcatcctgtcactgagtggatagctgaagtaaatttgcctgcggctcaagttgctgttggaatgggtatacccctttggcagattccagagatcaggcgcttctacggaatgaaccatggaggaggctatgacctttggaggaaaacagcagctctagcgactccatttaactttgatgaagtagattctaaatggccaaaaggccactgcgtagctgttagaataactagcgaggatccagatgatgggtttaagcctactggtggaaaagtaaaggagataagtttcaagagtaaaccaaatgtttgggcctatttctcagtaaagtctggtggaggcatccatgaattcgctgattctcagttcggacatgtttttgcgtatggaactactagatcggcagcaataactaccatggctcttgcactaaaagaggttcaaattcgtggagaaattcattcaaacgtagactacacagttgacctattaaatgcctcagattttagagaaaataagattcatactggttggctggataccaggatagccatgcgtgttcaagctgagaggcctccatggtatatttcagtcgttggaggggctttatataaaacagtaactgccaacacggccactgtttctgattatgttggttatcttaccaagggccagattccaccaaagcatatatcccttgtctatacgactgttgctttgaatatagatgggaaaaaatatacaatcgatactgtgaggagtggacatggtagctacagattgcgaatgaatggatcaacggttgacgcaaatgtacaaatattatgtgatggtgggcttttaatgcagctggatggaaacagccatgtaatttatgctgaagaagaggccagtggtacacgacttcttattgatggaaagacatgcatgttacagaatgaccatgacccatcaaagttattagctgagacaccatgcaaacttcttcgtttcttggttgctgatggtgctcatgttgatgctgatgtaccatatgcggaagttgaggttatgaagatgtgcatgcccctcttatcacccgcttctggtgtcatacatgttgtaatgtctgagggccaagcaatgcaggctggtgatcttatagctaggctggatcttgatgacccttctgctgttaagagagctgagccgttcgaagatacttttccacaaatgggtctccctattgctgcttctggccaagttcacaaattatgtgctgcaagtctgaatgcttgtcgaatgatccttgcggggtatgagcatgatattgacaaggttgtgccagagttggtatactgcctagacactccggagcttcctttcctgcagtgggaggagcttatgtctgttttagcaactagacttccaagaaatcttaaaagtgagttggagggcaaatatgaggaatacaaagtaaaatttgactctgggataatcaatgatttccctgccaatatgctacgagtgataattgaggaaaatcttgcatgtggttctgagaaggagaaggctacaaatgagaggcttgttgagcctcttatgagcctactgaagtcatatgagggtgggagagaaagtcatgctcactttgttgtcaagtccctttttgaggagtatctctatgttgaagaattgttcagtgatggaattcagtctgatgtgattgagcgtctgcgccttcaacatagtaaagacctacagaaggtcgtagacattgtgttgtcccaccagagtgttagaaataaaactaagctgatactaaaactcatggagagtctggtctatccaaatcctgctgcctacagggatcaattgattcgcttttcttcccttaatcacaaagcgtattacaagttggcacttaaagctagtgaacttcttgaacaaacaaaacttagtgagctccgtgcaagaatagcaaggagcctttcagagctggagatgtttactgaggaaagcaagggtctctccatgcataagcgagaaattgccattaaggagagcatggaagatttagtcactgctccactgccagttgaagatgcgctcatttctttatttgattgtagtgatacaactgttcaacagagagtgattgagacttatatagctcgattataccagcctcatcttgtaaaggacagtatcaaaatgaaatggatagaatcgggtgttattgctttatgggaatttcctgaagggcattttgatgcaagaaatggaggagcggttcttggtgacaaaagatggggtgccatggtcattgtcaagtctcttgaatcactttcaatggccattagatttgcactaaaggagacatcacactacactagctctgagggcaatatgatgcatattgctttgttgggtgctgataataagatgcatataattcaagaaagtggtgatgatgctgacagaatagccaaacttcccttgatactaaaggataatgtaaccgatctgcatgcctctggtgtgaaaacaataagtttcattgttcaaagagatgaagcacggatgacaatgcgtcgtaccttcctttggtctgatgaaaagctttcttatgaggaagagccaattctccggcatgtggaacctcctctttctgcacttcttgagttggacaagttgaaagtgaaaggatacaatgaaatgaagtataccccatcacgggatcgtcaatggcatatctacacacttagaaatactgaaaaccccaaaatgttgcaccgggtatttttccgaacccttgtcaggcaacccagtgtatccaacaagttttcttcgggccagattggtgacatggaagttgggagtgctgaagaacctctgtcatttacatcaaccagcatattaagatctttgatgactgctatagaggaattggagcttcacgcaattagaactggccattcacacatgtatttgcatgtattgaaagaacaaaagcttcttgatcttgttccagtttcagggaatacagttttggatgttggtcaagatgaagctactgcatattcacttttaaaagaaatggctatgaagatacatgaacttgttggtgcaagaatgcaccatctttctgtatgccaatgggaagtgaaacttaagttggactgcgatggtcctgccagtggtacctggaggattgtaacaaccaatgttactagtcacacttgcactgtggatatctaccgtgagatggaagataaagaatcacggaagttagtataccatcccgccactccggcggctggtcctctgcatggtgtggcactgaataatccatatcagcctttgagtgtcattgatctcaaacgctgttctgctaggaataatagaactacatactgctatgattttccactggcatttgaaactgcagtgaggaagtcatggtcctctagtacctctggtgcttctaaaggtgttgaaaatgcccaatgttatgttaaagctacagagttggtatttgcggacaaacatgggtcatggggcactcctttagttcaaatggaccggcctgctgggctcaatgacattggtatggtagcttggaccttgaagatgtccactcctgaatttcctagtggtagggagattattgttgttgcaaatgatattacgttcagagctggatcatttggcccaagggaagatgcattttttgaagctgttaccaacctagcctgtgagaagaaacttcctcttatttatttggcagcaaattctggtgctcgaattggcatagcagatgaagtgaaatcttgcttccgtgttgggtggtctgatgatggcagccctgaacgtgggtttcagtacatttatctaagcgaagaagactatgctcgtattggcacttctgtcatagcacataagatgcagctagacagtggtgaaattaggtgggttattgattctgttgtgggcaaggaagatggacttggtgtggagaatatacatggaagtgctgctattgccagtgcttattctagggcatataaggagacatttacacttacatttgtgactggaagaactgttggaataggagcttatcttgctcgacttggcatccggtgcatacagcgtcttgaccagcctattattcttacaggctattctgcactgaacaagcttcttgggcgggaagtgtacagctcccacatgcagttgggtggtcccaaaatcatggcaactaatggtgttgtccatcttactgtttcagatgaccttgaaggcgtttctaatatattgaggtggctcagttatgttcctgcctacattggtggaccacttccagtaacaacaccgttggacccaccggacagacctgttgcatacattcctgagaactcgtgtgatcctcgagcggctatccgtggtgttgatgacagccaagggaaatggttaggtggtatgtttgataaagacagctttgtggaaacatttgaaggttgggctaagacagtggttactggcagagcaaagcttggtggaattccagtgggtgtgatagctgtggagactcagaccatgatgcaaactatccctgctgaccctggtcagcttgattcccgtgagcaatctgttcctcgtgctggacaagtgtggtttccagattctgcaaccaagactgcgcaggcattgctggacttcaaccgtgaaggattacctctgttcatcctcgctaactggagaggcttctctggtggacaaagagatctttttgaaggaattcttcaggctggctcgactattgttgagaaccttaggacatacaatcagcctgcctttgtctacattcccatggctgcagagctacgaggaggggcttgggttgtggttgatagcaagataaacccagaccgcattgagtgctatgctgagaggactgcaaaaggcaatgttctggaaccgcaagggttaattgagatcaagttcaggtcagaggaactccaggattgcatgagtcggcttgacccaacattaattgatctgaaagcaaaactcgaagtagcaaataaaaatggaagtgctgacacaaaatcgcttcaagaaaatatagaagctcgaacaaaacagttgatgcctctatatactcagattgcgatacggtttgctgaattgcatgatacatccctcagaatggctgcgaaaggtgtgattaagaaagttgtggactgggaagaatcacgatctttcttctataagagattacggaggaggatctctgaggatgttcttgcaaaagaaattagagctgtagcaggtgagcagttttcccaccaaccagcaatcgagctgatcaagaaatggtattcagcttcacatgcagctgaatgggatgatgacgatgcttttgttgcttggatggataaccctgaaaactacaaggattatattcaatatcttaaggctcaaagagtatcccaatccctctcaagtctttcagattccagctcagatttgcaagccctgccacagggtctttccatgttactagataagatggatccctctagaagagctcaacttgttgaagaaatcaggaaggtccttggttga

SEQ ID NO: 7 - DNA, 25 bp, Artificial Sequence
  source: /note="Description of Artificial Sequence: Synthetic primer"
gcaaatgatattacgttcagagctg

SEQ ID NO: 8 - DNA, 24 bp, Artificial Sequence
  source: /note="Description of Artificial Sequence: Synthetic primer"
gttaccaacctagcctgtgagaag

SEQ ID NO: 9 - DNA, 26 bp, Artificial Sequence
  source: /note="Description of Artificial Sequence: Synthetic primer"
gatttcttcaacaagttgagctcttc

SEQ ID NO: 10 - DNA, 24 bp, Artificial Sequence
  source: /note="Description of Artificial Sequence: Synthetic primer"
agtaacatggaaagaccctgtggc

SEQ ID NO: 11 - DNA, 6978 bp, Zea mays
atgtcacagcttggattagccgcagctgcctcaaaggccttgccactactccctaatcgccagagaagttcagctgggactacattctcatcatcttcattatcgaggcccttaaacagaaggaaaagccgtactcgttcactccgtgatggcggagatggggtatcagatgccaaaaagcacagccagtctgttcgtcaaggtcttgctggcattatcgacctcccaagtgaggcaccttccgaagtggatatttcacatggatctgaggatcctagggggccaacagattcttatcaaatgaatgggattatcaatgaaacacataatggaagacatgcctcagtgtccaaggttgttgaattttgtgcggcactaggtggcaaaacaccaattcacagtatattagtggccaacaatggaatggcagcagcaaaatttatgaggagtgtccggacatgggctaatgatacttttggatctgagaaggcaattcaactcatagctatggcaactccggaagacatgaggataaatgcagaacacattagaattgctgaccaattcgtagaggtgcctggtggaacaaacaataataactacgccaatgttcaactcatagtggagatggcacaaaaactaggtgtttctgctgtttggcctggttggggtcatgcttctgagaatcctgaactgccagatgcattgaccgcaaaagggatcgtttttcttggcccacctgcatcatcaatgaatgctttgggagataaggtcggctcagctctcattgctcaagcagccggggtcccaactcttgctcggagtggatcacatgttgaagttccattagagtgctgcttagacgcgatacctgaggagatgtatagaaaagcttgcgttactaccacagaggaagcagttgcaagttgtcaagtggttggttatcctgccatgattaaggcatcctggggaggtggtggtaaaggaataagaaaggttcataatgatgatgaggttagagcgctgtttaagcaagtacaaggtgaagtccctggctccccaatatttgtcatgaggcttgcatcccagagtcggcatcttgaagttcagttgctttgtgatcaatatggtaatgtagcagcacttcacagtcgtgattgcagtgtgcaacggcgacaccagaagattattgaagaaggtccagttactgttgctcctcgtgagacagttaaagcacttgagcaggcagcaaggaggcttgctaaggctgtgggttatgttggtgctgctactgttgagtatctttacagcatggaaactggagactactattttctggaacttaatccccgactacaggttgagcatccagtcaccgagtggatagctgaagtaaatctgcctgcagctcaagttgctgttggaatgggcatacctctttggcagattccagaaatcagacgtttctatggaatggactatggaggagggtatgacatttggaggaaaacagcagctcttgctacaccatttaattttgatgaagtagattctcaatggccaaagggccattgtgtagcagttagaattactagtgaggacccagatgatggtttcaaacctactggtgggaaagtgaaggagataagttttaaaagcaagcctaatgtttgggcctacttctcagtaaagtctggtggaggcattcatgaatttgctgattctcagttcggacatgtttttgcatatgggctctctagatcagcagcaataacaaacatgactcttgcattaaaagagattcaaattcgtggagaaattcattcaaatgttgattacacagttgacctcttaaatgcttcagactttagagaaaacaagattcatactggttggctcgacaccagaatagctatgcgtgttcaagctgagaggcccccatggtatatttcagtggttggaggtgctttatataaaacagtaaccaccaatgcagccactgtttctgaatatgttagttatctcaccaagggccagattccaccaaagcatatatcccttgtcaattctacagttaatttgaatatagaagggagcaaatacacaattgaaactgtaaggactggacatggtagctacaggttgagaatgaatgattcaacagttgaagcgaatgtacaatctttatgtgatggtggcctcttaatgcagttggatggaaacagccatgtaatttatgcagaagaagaagctggtggtacacggcttcagattgatggaaagacatgtttattgcagaatgaccatgatccatcaaagttattagctgagacaccctgcaaacttcttcgtttcttggttgctgatggtgctcatgttgatgcggatgtaccatacgcggaagttgaggttatgaagatgtgcatgcctctcttgtcacctgcttctggtgtcattcattgtatgatgtctgagggccaggcattgcaggctggtgatcttatagcaaggttggatcttgatgacccttctgctgtgaaaagagctgagccatttgatggaatatttccacaaatggagctccctgttgctgtctctagtcaagtacacaaaagatatgctgcaagtttgaatgctgctcgaatggtccttgcaggatatgagcacaatattaatgaagtcgttcaagatttggtatgctgcctggacaaccctgagcttcctttcctacagtgggatgaacttatgtctgttctagcaacgaggcttccaagaaatctcaagagtgagttagaggataaatacaaggaatacaagttgaatttttaccatggaaaaaacgaggactttccatccaagttgctaagagacatcattgaggaaaatctttcttatggttcagagaaggaaaaggctacaaatgagaggcttgttgagcctcttatgaacctactgaagtcatatgagggtgggagagagagccatgcacattttgttgtcaagtctcttttcgaggagtatcttacagtggaagaactttttagtgatggcattcagtctgacgtgattgaaacattgcggcatcagcacagtaaagacctgcagaaggttgtagacattgtgttgtctcaccagggtgtgaggaacaaagctaagcttgtaacggcacttatggaaaagctggtttatccaaatcctggtggttacagggatctgttagttcgcttttcttccctcaatcataaaagatattataagttggcccttaaagcaagtgaacttcttgaacaaaccaaactaagtgaactccgtgcaagcgttgcaagaagcctttcggatctggggatgcataagggagaaatgagtattaaggataacatggaagatttagtctctgccccattacctgttgaagatgctctgatttctttgtttgattacagtgatcgaactgttcagcagaaagtgattgagacatacatatcacgattgtaccagcctcatcttgtaaaggatagcatccaaatgaaattcaaggaatctggtgctattactttttgggaattttatgaagggcatgttgatactagaaatggacatggggctattattggtgggaagcgatggggtgccatggtcgttctcaaatcacttgaatctgcgtcaacagccattgtggctgcattaaaggattcggcacagttcaacagctctgagggcaacatgatgcacattgcattattgagtgctgaaaatgaaagtaatataagtggaataagcagtgatgatcaagctcaacataagatggaaaagcttagcaagatactgaaggatactagcgttgcaagtgatctccaagctgctggtttgaaggttataagttgcattgttcaaagagatgaagctcgcatgccaatgcgccacacattcctctggttggatgacaagagttgttatgaagaagagcagattctccggcatgtggagcctcccctctctacacttcttgaattggataagttgaaggtgaaaggatacaatgaaatgaagtatactccttcgcgtgaccgccaatggcatatctacacactaagaaatactgaaaaccccaaaatgttgcatagggtgtttttccgaactattgtcaggcaacccaatgcaggcaacaagtttacatcggctcagatcagcgacgctgaagtaggatgtcccgaagaatctctttcatttacatcaaatagcatcttaagatcattgatgactgctattgaagaattagagcttcatgcaattaggacaggtcattctcacatgtatttgtgcatactgaaagagcaaaagcttcttgacctcattccattttcagggagtacaattgttgatgttggccaagatgaagctaccgcttgttcacttttaaaatcaatggctttgaagatacatgagcttgttggtgcaaggatgcatcatctgtctgtatgccagtgggaggtgaaactcaagttggactgtgatggccctgcaagtggtacctggagagttgtaactacaaatgttactggtcacacctgcaccattgatatataccgagaagtggaggaaatagaatcgcagaagttagtgtaccattcagccacttcgtcagctggaccattgcatggtgttgcactgaataatccatatcaacctttgagtgtgattgatctaaagcgctgctctgctaggaacaacagaacaacatattgctatgattttccgctggcctttgaaactgcactgcagaagtcatggcagtccaatggctctactgtttctgaaggcaatgaaaatagtaaatcctacgtgaaggcaactgagctagtgtttgctgaaaaacatgggtcctggggcactcctataattccgatggaacgccctgctgggctcaacgacattggtatggtcgcttggatcatggagatgtcaacacctgaatttcccaatggcaggcagattattgttgtagcaaatgatatcactttcagagctggatcatttggcccaagggaagatgcattttttgaaactgtcactaacctggcttgcgaaaggaaacttcctcttatatacttggcagcaaactctggtgctaggattggcatagctgatgaagtaaaatcttgcttccgtgttggatggtctgacgaaggcagtcctgaacgagggtttcagtacatctatctgactgaagaagactatgctcgcattagctcttctgttatagcacataagctggagctagatagtggtgaaattaggtggattattgactctgttgtgggcaaggaggatgggcttggtgtcgagaacatacatggaagtgctgctattgccagtgcttattctagggcatatgaggagacatttacacttacatttgtgactgggcggactgtaggaataggagcttatcttgctcgacttggtatacggtgcatacagcgtcttgaccagcctattattttaacagggttttctgccctgaacaagctccttgggcgggaagtgtacagctcccacatgcagcttggtggtcctaagatcatggcgactaatggtgttgtccacctcactgttccagatgaccttgaaggtgtttccaatatattgaggtggctcagctatgttcctgcaaacattggtggacctcttcctattaccaaacctctggaccctccagacagacctgttgcttacatccctgagaacacatgcgatccacgtgcagctatctgtggtgtagatgacagccaagggaaatggttgggtggtatgtttgacaaagacagctttgtggagacatttgaaggatgggcaaaaacagtggttactggcagagcaaagcttggaggaattcctgtgggcgtcatagctgtggagacacagaccatgatgcagatcatccctgctgatccaggtcagcttgattcccatgagcgatctgtccctcgtgctggacaagtgtggttcccagattctgcaaccaagaccgctcaggcattattagacttcaaccgtgaaggattgcctctgttcatcctggctaattggagaggcttctctggtggacaaagagatctctttgaaggaattcttcaggctgggtcaacaattgtcgagaaccttaggacatctaatcagcctgcttttgtgtacattcctatggctggagagcttcgtggaggagcttgggttgtggtcgatagcaaaataaatccagaccgcattgagtgttatgctgaaaggactgccaaaggtaatgttctcgaacctcaagggttaattgaaatcaagttcaggtcagaggaactccaagactgtatgggtaggcttgacccagagttgataaatctgaaagcaaaactccaagatgtaaatcatggaaatggaagtctaccagacatagaagggattcggaagagtatagaagcacgtacgaaacagttgctgcctttatatacccagattgcaatacggtttgctgaattgcatgatacttccctaagaatggcagctaaaggtgtgattaagaaagttgtagactgggaagaatcacgctcgttcttctataaaaggctacggaggaggatcgcagaagatgttcttgcaaaagaaataaggcagatagtcggtgataaatttacgcaccaattagcaatggagctcatcaaggaatggtaccttgcttctcaggccacaacaggaagcactggatgggatgacgatgatgcttttgttgcctggaaggacagtcctgaaaactacaaggggcatatccaaaagcttagggctcaaaaagtgtctcattcgctctctgatcttgctgactccagttcagatctgcaagcattctcgcagggtctttctacgctattagataagatggatccctctcagagagcgaagtttgttcaggaagtcaagaaggtccttgattga

SEQ ID NO: 12 - protein, 2325 aa, Zea mays
MSQLGLAAAASKALPLLPNRQRSSAGTTFSSSSLSRPLNRRKSRTRSLRDGGDGVSDAKKHSQSVRQGLAGIIDLPSEAPSEVDISHGSEDPRGPTDSYQMNGIINETHNGRHASVSKVVEFCAALGGKTPIHSILVANNGMAAAKFMRSVRTWANDTFGSEKAIQLIAMATPEDMRINAEHIRIADQFVEVPGGTNNNNYANVQLIVEMAQKLGVSAVWPGWGHASENPELPDALTAKGIVFLGPPASSMNALGDKVGSALIAQAAGVPTLARSGSHVEVPLECCLDAIPEEMYRKACVTTTEEAVASCQVVGYPAMIKASWGGGGKGIRKVHNDDEVRALFKQVQGEVPGSPIFVMRLASQSRHLEVQLLCDQYGNVAALHSRDCSVQRRHQKIIEEGPVTVAPRETVKALEQAARRLAKAVGYVGAATVEYLYSMETGDYYFLELNPRLQVEHPVTEWIAEVNLPAAQVAVGMGIPLWQIPEIRRFYGMDYGGGYDIWRKTAALATPFNFDEVDSQWPKGHCVAVRITSEDPDDGFKPTGGKVKEISFKSKPNVWAYFSVKSGGGIHEFADSQFGHVFAYGLSRSAAITNMTLALKEIQIRGEIHSNVDYTVDLLNASDFRENKIHTGWLDTRIAMRVQAERPPWYISVVGGALYKTVTTNAATVSEYVSYLTKGQIPPKHISLVNSTVNLNIEGSKYTIETVRTGHGSYRLRMNDSTVEANVQSLCDGGLLMQLDGNSHVIYAEEEAGGTRLQIDGKTCLLQNDHDPSKLLAETPCKLLRFLVADGAHVDADVPYAEVEVMKMCMPLLSPASGVIHCMMSEGQALQAGDLIARLDLDDPSAVKRAEPFDGIFPQMELPVAVSSQVHKRYAASLNAARMVLAGYEHNINEVVQDLVCCLDNPELPFLQWDELMSVLATRLPRNLKSELEDKYKEYKLNFYHGKNEDFPSKLLRDIIEENLSYGSEKEKATNERLVEPLMNLLKSYEGGRESHAHFVVKSLFEEYLTVEELFSDGIQSDVIETLRHQHSKDLQKVVDIVLSHQGVRNKAKLVTALMEKLVYPNPGGYRDLLVRFSSLNHKRYYKLALKASELLEQTKLSELRASVARSLSDLGMHKGEMSIKDNMEDLVSAPLPVEDALISLFDYSDRTVQQKVIETYISRLYQPHLVKDSIQMKFKESGAITFWEFYEGHVDTRNGHGAIIGGKRWGAMVVLKSLESASTAIVAALKDSAQFNSSEGNMMHIALLSAENESNISGISSDDQAQHKMEKLSKILKDTSVASDLQAAGLKVISCIVQRDEARMPMRHTFLWLDDKSCYEEEQILRHVEPPLSTLLELDKLKVKGYNEMKYTPSRDRQWHIYTLRNTENPKMLHRVFFRTIVRQPNAGNKFTSAQISDAEVGCPEESLSFTSNSILRSLMTAIEELELHAIRTGHSHMYLCILKEQKLLDLIPFSGSTIVDVGQDEATACSLLKSMALKIHELVGARMHHLSVCQWEVKLKLDCDGPASGTWRVVTTNVTGHTCTIDIYREVEEIESQKLVYHSATSSAGPLHGVALNNPYQPLSVIDLKRCSARNNRTTYCYDFPLAFETALQKSWQSNGSTVSEGNENSKSYVKATELVFAEKHGSWGTPIIPMERPAGLNDIGMVAWIMEMSTPEFPNGRQIIVVANDITFRAGSFGPREDAFFETVTNLACERKLPLIYLAANSGARIGIADEVKSCFRVGWSDEGSPERGFQYIYLTEEDYARISSSVIAHKLELDSGEIRWIIDSVVGKEDGLGVENIHGSAAIASAYSRAYEETFTLTFVTGRTVGIGAYLARLGIRCIQRLDQPIILTGFSALNKLLGREVYSSHMQLGGPKIMATNGVVHLTVPDDLEGVSNILRWLSYVPANIGGPLPITKPLDPPDRPVAYIPENTCDPRAAICGVDDSQGKWLGGMFDKDSFVETFEGWAKTVVTGRAKLGGIPVGVIAVETQTMMQIIPADPGQLDSHERSVPRAGQVWFPDSATKTAQALLDFNREGLPLFILANWRGFSGGQRDLFEGILQAGSTIVENLRTSNQPAFVYIPMAGELRGGAWVVVDSKINPDRIECYAERTAKGNVLEPQGLIEIKFRSEELQDCMGRLDPELINLKAKLQDVNHGNGSLPDIEGIRKSIEARTKQLLPLYTQIAIRFAELHDTSLRMAAKGVIKKVVDWEESRSFFYKRLRRRIAEDVLAKEIRQIVGDKFTHQLAMELIKEWYLASQATTGSTGWDDDDAFVAWKDSPENYKGHIQKLRAQKVSHSLSDLADSSSDLQAFSQGLSTLLDKMDPSQRAKFVQEVKKVLD

SEQ ID NO: 13 - DNA, 6975 bp, Zea mays
atgtcacagcttggattagccgcagctgcctcaaaggccttgccactactccctaatcgccagagaagttcagctgggactacattctcatcatcttcattatcgaggcccttaaacagaaggaaaagccgtactcgttcactccgtgatggcggagatggggtatcagatgccaaaaagcacagccagtctgttcgtcaaggtcttgctggcattatcgacctcccaagtgaggcaccttccgaagtggatatttcacatggatctgaggatcctagggggccaacagattcttatcaaatgaatgggattatcaatgaaacacataatggaagacatgcctcagtgtccaaggttgttgaattttgtgcggcactaggtggcaaaacaccaattcacagtatattagtggccaacaatggaatggcagcagcaaaatttatgaggagtgtccggacatgggctaatgatacttttggatctgagaaggcaattcaactcatagctatggcaactccggaagacatgaggataaatgcagaacacattagaattgctgaccaattcgtagaggtgcctggtggaacaaacaataataactacgccaatgttcaactcatagtggagatggcacaaaaactaggtgtttctgctgtttggcctggttggggtcatgcttctgagaatcctgaactgccagatgcattgaccgcaaaagggatcgtttttcttggcccacctgcatcatcaatgaatgctttgggagataaggtcggctcagctctcattgctcaagcagccggggtcccaactcttgcttggagtggatcacatgttgaagttccattagagtgctgcttagacgcgatacctgaggagatgtatagaaaagcttgcgttactaccacagaggaagcagttgcaagttgtcaagtggttggttatcctgccatgattaaggcatcctggggaggtggtggtaaaggaataagaaaggttcataatgatgatgaggttagagcgctgtttaagcaagtacaaggtgaagtccctggctccccaatatttgtcatgaggcttgcatcccagagtcggcatcttgaagttcagttgctttgtgatcaatatggtaatgtagcagcacttcacagtcgtgattgcagtgtgcaacggcgacaccagaagattattgaagaaggtccagttactgttgctcctcgtgagacagttaaagcacttgagcaggcagcaaggaggcttgctaaggctgtgggttatgttggtgctgctactgttgagtatctttacagcatggaaactggagactactattttctggaacttaatccccgactacaggttgagcatccagtcaccgagtggatagctgaagtaaatctgcctgcagctcaagttgctgttggaatgggcatacctctttggcagattccagaaatcagacgtttctatggaatggactatggaggagggtatgacatttggaggaaaacagcagctcttgctacaccatttaattttgatgaagtagattctcaatggccaaagggccattgtgtagcagttagaattactagtgaggacccagatgatggtttcaaacctactggtgggaaagtgaaggagataagttttaaaagcaagcctaatgtttgggcctacttctcagtaaagtctggtggaggcattcatgaatttgctgattctcagttcggacatgtttttgcatatgggctctctagatcagcagcaataacaaacatgactcttgcattaaaagagattcaaattcgtggagaaattcattcaaatgttgattacacagttgacctcttaaatgcttcagactttagagaaaacaagattcatactggttggctcgacaccagaatagctatgcgtgttcaagctgagaggcccccatggtatatttcagtggttgggggtgctttatataaaacagtaaccaccaatgcagccactgtttctgaatatgttagttatctcaccaagggccagattccaccaaagcatatatcccttgtcaattctacagttaatttgaatatagaagggagcaaatacacaattgaaactgtaaggactggacatggtagctacaggttgagaatgaatgattcaacagttgaagcgaatgtacaatctttatgtgatggtggcctcttaatgcagttggatggaaacagccatgtaatttatgcagaagaagaagctggtggtacacggcttcagattgatggaaagacatgtttattgcagaatgaccatgatccatcaaagttattagctgagacaccctgcaaacttcttcgtttcttggttgctgatggtgctcatgttgatgcggatgtaccatacgcggaagttgaggttatgaagatgtgcatgcctctcttgtcgcctgcttctggtgtcattcattgtatgatgtctgagggccaggcattgcaggctggtgatcttatagcaaggttggatcttgatgacccttctgctgtgaaaagagctgagccatttgatggaatatttccacaaatggagctccctgttgctgtctctagtcaagtacacaaaagatatgctgcaagtttgaatgctgctcgaatggtccttgcaggatatgagcacaatattaatgaagtcgttcaagatttggtatgctgcctggacaaccctgagcttcctttcctacagtgggatgaacttatgtctgttctagcaacgaggcttccaagaaatctcaagagtgagttagaggataaatacaaggaatacaagttgaatttttaccatggaaaaaacgaggactttccatccaagttgctaagagacatcattgaggaaaatctttcttatggttcagagaaggaaaaggctacaaatgagaggcttgttgagcctcttatgaacctactgaagtcatatgagggtgggagagagagccatgcacattttgttgtcaagtctcttttcgaggagtatcttacagtggaagaactttttagtgatggcattcagtctgacgtgattgaaacattgcggcatcagcacagtaaagacctgcagaaggttgtagacattgtgttgtctcaccagggtgtgaggaacaaagctaagcttgtaacggcacttatggaaaagctggtttatccaaatcctggtggttacagggatctgttagttcgcttttcttccctcaatcataaaagatattataagttggcccttaaagcaagtgaacttcttgaacaaaccaaactaagtgaactccgtgcaagcgttgcaagaagcctttcggatctggggatgcataagggagaaatgagtattaaggataacatggaagatttagtctctgccccattacctgttgaagatgctctgatttctttgtttgattacagtgatcgaactgttcagcagaaagtgattgagacatacatatcacgattgtaccagcctcatcttgtaaaggatagcatccaaatgaaattcaaggaatctggtgctattactttttgggaattttatgaagggcatgttgatactagaaatggacatggggctattattggtgggaagcgatggggtgccatggtcgttctcaaatcacttgaatctgcgtcaacagccattgtggctgcattaaaggattcggcacagttcaacagctctgagggcaacatgatgcacattgcattattgagtgctgaaaatgaaagtaatataagtggaataagtgatgatcaagctcaacataagatggaaaagcttagcaagatactgaaggatactagcgttgcaagtgatctccaagctgctggtttgaaggttataagttgcattgttcaaagagatgaagctcgcatgccaatgcgccacacattcctctggttggatgacaagagttgttatgaagaagagcagattctccggcatgtggagcctcccctctctacacttcttgaattggataagttgaaggtgaaaggatacaatgaaatgaagtatactccttcgcgtgaccgccaatggcatatctacacactaagaaatactgaaaaccccaaaatgttgcatagggtgtttttccgaactattgtcaggcaacccaatgcaggcaacaagtttacatcggctcagatcagcgacgctgaagtaggatgtcccgaagaatctctttcatttacatcaaatagcatcttaagatcattgatgactgctattgaagaattagagcttcatgcaattaggacaggtcattctcacatgtatttgtgcatactgaaagagcaaaagcttcttgacctcattccattttcagggagtacaattgttgatgttggccaagatgaagctaccgcttgttcacttttaaaatcaatggctttgaagatacatgagcttgttggtgcaaggatgcatcatctgtctgtatgccagtgggaggtgaaactcaagttggactgtgatggccctgcaagtggtacctggagagttgtaactacaaatgttactggtcacacctgcaccattgatatataccgagaagtggaggaaatagaatcgcagaagttagtgtaccattcagccacttcgtcagctggaccattgcatggtgttgcactgaataatccatatcaacctttgagtgtgattgatctaaagcgctgctctgctaggaacaacagaacaacatattgctatgattttccgctggcctttgaaactgcactgcagaagtcatggcagaccaatggctctactgtttctgaaggcaatgaaaatagtaaatcctacgtgaaggcaactgagctagtgtttgctgaaaaacatgggtcctggggcactcctataattccgatggaacgccctgctgggctcaacgacattggtatggtcgcttggatcatggagatgtcaacacctgaatttcccaatggcaggcagattattgttgtagcaaatgatatcactttcagagctggatcatttggcccaagggaagatgcattttttgaaactgtcactaacctggcttgcgaaaggaaacttcctcttatatacttggcagcaaactctggtgctaggattggcatagctgatgaagtaaaatcttgcttccgtgttggatggtctgacgaaggcagtcctgaacgagggtttcagtacatctatctgactgaagaagactatgctcgcattagctcttctgttatagcacataagctggagctagatagtggtgaaattaggtggattattgactctgttgtgggcaaggaggatgggcttggtgtcgagaacatacatggaagtgctgctattgccagtgcttattctagggcatatgaggagacatttacacttacatttgtgactgggcggactgtaggaataggagcttatcttgctcgacttggtatacggtgcatacagcgtcttgaccagcctattattttaacagggttttctgccctgaacaagctccttgggcgggaagtgtacagctcccacatgcagcttggtggtcctaagatcatggcgactaatggtgttgtccacctcactgttccagatgaccttgaaggtgtttccaatatattgaggtggctcagctatgttcctgcaaacattggtggacctcttcctattaccaaacctctggaccctccagacagacctgttgcttacatccctgagaacacatgcgatccacgtgcagctatctgtggtgtagatgacagccaagggaaatggttgggtggtatgtttgacaaagacagctttgtggagacatttgaaggatgggcaaaaacagtggttactggcagagcaaagcttggaggaattcctgtgggcgtcatagctgtggagacacagaccatgatgcagatcatccctgctgatccaggtcagcttgattcccatgagcgatctgtccctcgtgctggacaagtgtggttcccagattctgcaaccaagaccgctcaggcattattagacttcaaccgtgaaggattgcctctgttcatcctggctaattggagaggcttctctggtggacaaagagatctctttgaaggaattcttcaggctgggtcaacaattgtcgagaaccttaggacatataatcagcctgcttttgtgtacattcctatggctggagagcttcgtggaggagcttgggttgtggtcgatagcaaaataaatccagaccgcattgagtgttatgctgaaaggactgccaaaggtaatgttctcgaacctcaagggttaattgaaatcaagttcaggtcagaggaactccaagactgtatgggtaggcttgacccagagttgataaatctgaaagcaaaactccaagatgtaaatcatggaaatggaagtctaccagacatagaagggattcggaagagtatagaagcacgtacgaaacagttgctgcctttatatacccagattgcaatacggtttgctgaattgcatgatacttccctaagaatggcagctaaaggtgtgattaagaaagttgtagactgggaagaatcacgctcgttcttctataaaaggctacggaggaggatcgcagaagatgttcttgcaaaagaaataaggcagatagtcggtgataaatttacgcaccaattagcaatggagctcatcaaggaatggtaccttgcttctcaggccacaacaggaagcactggatgggatgacgatgatgcttttgttgcctggaaggacagtcctgaaaactacaaggggcatatccaaaagcttagggctcaaaaagtgtctcattcgctctctgatcttgctgactccagttcagatctgcaagcattctcgcagggtctttctacgctattagataagatggatccctctcagagagcgaagtttgttcaggaagtcaagaaggtccttgattga

SEQ ID NO: 14 - protein, 2324 aa, Zea mays
MSQLGLAAAASKALPLLPNRQRSSAGTTFSSSSLSRPLNRRKSRTRSLRDGGDGVSDAKKHSQSVRQGLAGIIDLPSEAPSEVDISHGSEDPRGPTDSYQMNGIINETHNGRHASVSKVVEFCAALGGKTPIHSILVANNGMAAAKFMRSVRTWANDTFGSEKAIQLIAMATPEDMRINAEHIRIADQFVEVPGGTNNNNYANVQLIVEMAQKLGVSAVWPGWGHASENPELPDALTAKGIVFLGPPASSMNALGDKVGSALIAQAAGVPTLAWSGSHVEVPLECCLDAIPEEMYRKACVTTTEEAVASCQVVGYPAMIKASWGGGGKGIRKVHNDDEVRALFKQVQGEVPGSPIFVMRLASQSRHLEVQLLCDQYGNVAALHSRDCSVQRRHQKIIEEGPVTVAPRETVKALEQAARRLAKAVGYVGAATVEYLYSMETGDYYFLELNPRLQVEHPVTEWIAEVNLPAAQVAVGMGIPLWQIPEIRRFYGMDYGGGYDIWRKTAALATPFNFDEVDSQWPKGHCVAVRITSEDPDDGFKPTGGKVKEISFKSKPNVWAYFSVKSGGGIHEFADSQFGHVFAYGLSRSAAITNMTLALKEIQIRGEIHSNVDYTVDLLNASDFRENKIHTGWLDTRIAMRVQAERPPWYISVVGGALYKTVTTNAATVSEYVSYLTKGQIPPKHISLVNSTVNLNIEGSKYTIETVRTGHGSYRLRMNDSTVEANVQSLCDGGLLMQLDGNSHVIYAEEEAGGTRLQIDGKTCLLQNDHDPSKLLAETPCKLLRFLVADGAHVDADVPYAEVEVMKMCMPLLSPASGVIHCMMSEGQALQAGDLIARLDLDDPSAVKRAEPFDGIFPQMELPVAVSSQVHKRYAASLNAARMVLAGYEHNINEVVQDLVCCLDNPELPFLQWDELMSVLATRLPRNLKSELEDKYKEYKLNFYHGKNEDFPSKLLRDIIEENLSYGSEKEKATNERLVEPLMNLLKSYEGGRESHAHFVVKSLFEEYLTVEELFSDGIQSDVIETLRHQHSKDLQKVVDIVLSHQGVRNKAKLVTALMEKLVYPNPGGYRDLLVRFSSLNHKRYYKLALKASELLEQTKLSELRASVARSLSDLGMHKGEMSIKDNMEDLVSAPLPVEDALISLFDYSDRTVQQKVIETYISRLYQPHLVKDSIQMKFKESGAITFWEFYEGHVDTRNGHGAIIGGKRWGAMVVLKSLESASTAIVAALKDSAQFNSSEGNMMHIALLSAENESNISGISDDQAQHKMEKLSKILKDTSVASDLQAAGLKVISCIVQRDEARMPMRHTFLWLDDKSCYEEEQILRHVEPPLSTLLELDKLKVKGYNEMKYTPSRDRQWHIYTLRNTENPKMLHRVFFRTIVRQPNAGNKFTSAQISDAEVGCPEESLSFTSNSILRSLMTAIEELELHAIRTGHSHMYLCILKEQKLLDLIPFSGSTIVDVGQDEATACSLLKSMALKIHELVGARMHHLSVCQWEVKLKLDCDGPASGTWRVVTTNVTGHTCTIDIYREVEEIESQKLVYHSATSSAGPLHGVALNNPYQPLSVIDLKRCSARNNRTTYCYDFPLAFETALQKSWQTNGSTVSEGNENSKSYVKATELVFAEKHGSWGTPIIPMERPAGLNDIGMVAWIMEMSTPEFPNGRQIIVVANDITFRAGSFGPREDAFFETVTNLACERKLPLIYLAANSGARIGIADEVKSCFRVGWSDEGSPERGFQYIYLTEEDYARISSSVIAHKLELDSGEIRWIIDSVVGKEDGLGVENIHGSAAIASAYSRAYEETFTLTFVTGRTVGIGAYLARLGIRCIQRLDQPIILTGFSALNKLLGREVYSSHMQLGGPKIMATNGVVHLTVPDDLEGVSNILRWLSYVPANIGGPLPITKPLDPPDRPVAYIPENTCDPRAAICGVDDSQGKWLGGMFDKDSFVETFEGWAKTVVTGRAKLGGIPVGVIAVETQTMMQIIPADPGQLDSHERSVPRAGQVWFPDSATKTAQALLDFNREGLPLFILANWRGFSGGQRDLFEGILQAGSTIVENLRTYNQPAFVYIPMAGELRGGAWVVVDSKINPDRIECYAERTAKGNVLEPQGLIEIKFRSEELQDCMGRLDPELINLKAKLQDVNHGNGSLPDIEGIRKSIEARTKQLLPLYTQIAIRFAELHDTSLRMAAKGVIKKVVDWEESRSFFYKRLRRRIAEDVLAKEIRQIVGDKFTHQLAMELIKEWYLASQATTGSTGWDDDDAFVAWKDSPENYKGHIQKLRAQKVSHSLSDLADSSSDLQAFSQGLSTLLDKMDPSQRAKFVQEVKKVLD

SEQ ID NO: 15 - DNA, 6936 bp, Triticum aestivum
atgggatccacacatttgcccattgtcggccttaatgcctcgacaacaccatcgctatccactattcgcccggtaaattcagccggtgctgcattccaaccatctgccccttctagaacctccaagaagaaaagtcgtcgtgttcagtcattaagggatggaggcgatggaggcgtgtcagaccctaaccagtctattcgccaaggtcttgccggcatcattgacctcccaaaggagggcacatcagctccggaagtggatatttcacatgggtccgaagaacccaggggctcctaccaaatgaatgggatactgaatgaagcacataatgggaggcatgcttcgctgtctaaggttgtcgaattttgtatggcattgggcggcaaaacaccaattcacagtgtattagttgcgaacaatggaatggcagcagctaagttcatgcggagtgtccgaacatgggctaatgaaacatttgggtcagagaaggcaattcagttgatagctatggctactccagaagacatgaggataaatgcagagcacattagaattgctgatcaatttgttgaagtacccggtggaacaaacaataacaactatgcaaatgtccaactcatagtggagatagcagtgagaaccggtgtttctgctgtttggcctggttggggccatgcatctgagaatcctgaacttccagatgcactaaatgcaaacggaattgtttttcttgggccaccatcatcatcaatgaacgcactaggtgacaaggttggttcagctctcattgctcaagcagcaggggttccgactcttccttggagtggatcacaggtggaaattccattagaagtttgtttggactcgatacccgcggagatgtataggaaagcttgtgttagtactacggaggaagcacttgcgagttgtcagatgattgggtatcccgccatgattaaagcatcatggggtggtggtggtaaagggatccgaaaggttaataatgacgatgatgtcagagcactgtttaagcaagtgcaaggtgaagttcctggctccccaatatttatcatgagacttgcatctcagagtcgacatcttgaagttcagttgctttgtgatcaatatggcaatgtagctgcgcttcacagtcgtgactgcagtgtgcaacggcgacaccaaaagattattgaggaaggaccagttactgttgctcctcgcgagacagtgaaagagctagagcaagcagcaaggaggcttgctaaggctgtgggttatgttggtgctgctactgttgaatatctctacagcatggagactggtgaatactattttctggaacttaatccacggttgcaggttgagcatccagtcaccgagtggatagctgaagtaaacttgcctgcagctcaagttgcagttggaatgggtatacccctttggcaggttccagagatcagacgtttctatggaatggacaatggaggaggctatgacatttggaggaaaacagcagctcttgctactccatttaacttcgatgaagtggattctcaatggccaaagggtcattgtgtagcagttaggataaccagtgaggatccagatgacggattcaagcctaccggtggaaaagtaaaggagatcagttttaaaagcaagccaaatgtttgggcctatttctctgttaagtccggtggaggcattcatgaatttgctgattctcagtttggacatgtttttgcatatggagtgtctagagcagcagcaataaccaacatgtctcttgcgctaaaagagattcaaattcgtggagaaattcattcaaatgttgattacacagttgatctcttgaatgcctcagacttcaaagaaaacaggattcatactggctggctggataacagaatagcaatgcgagtccaagctgagagacctccgtggtatatttcagtggttggaggagctctatataaaacaataacgagcaacacagacactgtttctgaatatgttagctatctcgtcaagggtcagattccaccgaagcatatatcccttgtccattcaactgtttctttgaatatagaggaaagcaaatatacaattgaaactataaggagcggacagggtagctacagattgcgaatgaatggatcagttattgaagcaaatgtccaaacattatgtgatggtggacttttaatgcagttggatggaaacagccatgtaatttatgctgaagaagaggccggtggtacacggcttctaattgatggaaagacatgcttgttacagaatgatcacgatccttcaaggttattagctgagacaccctgcaaacttcttcgtttcttggttgccgatggtgctcatgttgaagctgatgtaccatatgcggaagttgaggttatgaagatgtgcatgcccctcttgtcacctgctgctggtgtcattaatgttttgttgtctgagggccagcctatgcaggctggtgatcttatagcaagacttgatcttgatgacccttctgctgtgaagagagctgagccatttaacggatctttcccagaaatgagccttcctattgctgcttctggccaagttcacaaaagatgtgccacaagcttgaatgctgctcggatggtccttgcaggatatgatcacccgatcaacaaagttgtacaagatctggtatcctgtctagatgctcctgagcttcctttcctacaatgggaagagcttatgtctgttttagcaactagacttccaaggcttcttaagagcgagttggagggtaaatacagtgaatataagttaaatgttggccatgggaagagcaaggatttcccttccaagatgctaagagagataatcgaggaaaatcttgcacatggttctgagaaggaaattgctacaaatgagaggcttgttgagcctcttatgagcctactgaagtcatatgagggtggcagagaaagccatgcacactttattgtgaagtcccttttcgaggactatctctcggttgaggaactattcagtgatggcattcagtctgatgtgattgaacgcctgcgccaacaacatagtaaagatctccagaaggttgtagacattgtgttgtctcaccagggtgtgagaaacaaaactaagctgatactaacactcatggagaaactggtctatccaaaccctgctgtctacaaggatcagttgactcgcttttcctccctcaatcacaaaagatattataagttggcccttaaagctagcgagcttcttgaacaaaccaagcttagtgagctccgcacaagcattgcaaggagcctttcagaacttgagatgtttactgaagaaaggacggccattagtgagatcatgggagatttagtgactgccccactgccagttgaagatgcactggtttctttgtttgattgtagtgatcaaactcttcagcagagggtgatcgagacgtacatatctcgattataccagcctcatcttgtcaaggatagtatccagctgaaatatcaggaatctggtgttattgctttatgggaattcgctgaagcgcattcagagaagagattgggtgctatggttattgtgaagtcgttagaatctgtatcagcagcaattggagctgcactaaagggtacatcacgctatgcaagctctgagggtaacataatgcatattgctttattgggtgctgataatcaaatgcatggaactgaagacagtggtgataacgatcaagctcaagtcaggatagacaaactttctgcgacactggaacaaaatactgtcacagctgatctccgtgctgctggtgtgaaggttattagttgcattgttcaaagggatggagcactcatgcctatgcgccataccttcctcttgtcggatgaaaagctttgttatgaggaagagccggttctccggcatgtggagcctcctctttctgctcttcttgagttgggtaagttgaaagtgaaaggatacaatgaggtgaagtatacaccgtcacgtgatcgtcagtggaacatatacacacttagaaatacagagaaccccaaaatgttgcacagggtgtttttccgaactcttgtcaggcaacccggtgcttccaacaaattcacatcaggcaacatcagtgatgttgaagtgggaggagctgaggaatctctttcatttacatcgagcagcatattaagatcgctgatgactgctatagaagagttggagcttcacgcgattaggacaggtcactctcatatgtttttgtgcatattgaaagagcaaaagcttcttgatcttgttcccgtttcagggaacaaagttgtggatattggccaagatgaagctactgcatgcttgcttctgaaagaaatggctctacagatacatgaacttgtgggtgcaaggatgcatcatctttctgtatgccaatgggaggtgaaacttaagttggacagcgatgggcctgccagtggtacctggagagttgtaacaaccaatgttactagtcacacctgcactgtggatatctaccgtgaggtcgaagatacagaatcacagaaactagtgtaccactctgctccatcgtcatctggtcctttgcatggcgttgcactgaatactccatatcagcctttgagtgttattgatctgaaacgttgctccgctagaaataacagaactacatactgctatgattttccgttggcatttgaaactgcagtgcagaagtcatggtctaacatttctagtgacactaaccgatgttatgttaaagcgacggagctggtgtttgctcacaagaacgggtcatggggcactcctgtaattcctatggagcgtcctgctgggctcaatgacattggtatggtagcttggatcttggacatgtccactcctgaatatcccaatggcaggcagattgttgtcatcgcaaatgatattacttttagagctggatcgtttggtccaagggaagatgcattttttgaaactgttaccaacctagcttgtgagaggaagcttcctctcatctacttggcagcaaactctggtgctcggatcggcatagcagatgaagtaaaatcttgcttccgtgttggatggtctgatgatggcagccctgaacgtgggtttcaatatatttatctgactgaagaagaccatgctcgtattagcgcttctgttatagcgcacaagatgcagcttgataatggtgaaattaggtgggttattgattctgttgtagggaaggaggatgggctaggtgtggagaacatacatggaagtgctgctattgccagtgcctattctagggcctatgaggagacatttacgcttacatttgtgactggaaggactgttggaataggagcatatcttgctcgacttggcatacggtgcatacagcgtactgaccagcccattatcctaactgggttctctgccttgaacaagcttcttggccgggaagtttacagctcccacatgcagttgggtggccccaaaattatggcgacaaacggtgttgtccatctgacagtttcagatgaccttgaaggtgtatctaatatattgaggtggctcagctatgttcctgccaacattggtggacctcttcctattacaaaatctttggacccacctgacagacccgttgcttacatccctgagaatacatgcgatcctcgtgctgccatcagtggcattgatgatagccaagggaaatggttggggggcatgttcgacaaagacagttttgtggagacatttgaaggatgggcgaagtcagttgttactggcagagcgaaactcggagggattccggtgggtgttatagctgtggagacacagactatgatgcagctcatccctgctgatccaggccagcttgattcccatgagcgatctgttcctcgtgctgggcaagtctggtttccagattcagctactaagacagcgcaggcaatgctggacttcaaccgtgaaggattacctctgttcatccttgctaactggagaggcttctctggtggacaaagagatctttttgaaggaatccttcaggctgggtcaacaattgttgagaaccttaggacatacaatcagcctgcctttgtatatatccccaaggctgcagagctacgtggaggggcttgggtcgtgattgatagcaagataaatccagatcgcattgagttctatgctgagaggactgcaaagggcaatgttctcgaacctcaagggttgatcgagatcaagttcaggtcagaggaactccaagagtgcatgggtaggcttgatccagaattgataaatctgaaggcaaagctccagggagtaaagcatgaaaatggaagtctacctgagtcagaatcccttcagaagagcatagaagcccggaagaaacagttgttgcctttgtatactcaaattgcggtacggttcgctgaattgcatgacacttcccttagaatggctgctaagggtgtgattaagaaggttgtagactgggaagattctaggtcgttcttctacaagagattacggaggaggatatccgaggatgttcttgcgaaggaaattagaggtgtaagtggcaagcagttttctcaccaatcggcaatcgagctgatccagaaatggtacttggcctctaagggagctgaaacaggaagcactgaatgggatgatgacgatgcttttgttgcctggagggaaaaccctgaaaactaccaggagtatatcaaagaactcagggctcaaagggtatctcagttgctctcagatgttgcagactccagtccagatctagaagccttgccacagggtctttctatgctattagagaagatggatccctcaaggagagcacagtttgttgaggaagtcaagaaagtccttaaatga

SEQ ID NO: 16 - protein, 2311 aa, Triticum aestivum
MGSTHLPIVGLNASTTPSLSTIRPVNSAGAAFQPSAPSRTSKKKSRRVQSLRDGGDGGVSDPNQSIRQGLAGIIDLPKEGTSAPEVDISHGSEEPRGSYQMNGILNEAHNGRHASLSKVVEFCMALGGKTPIHSVLVANNGMAAAKFMRSVRTWANETFGSEKAIQLIAMATPEDMRINAEHIRIADQFVEVPGGTNNNNYANVQLIVEIAVRTGVSAVWPGWGHASENPELPDALNANGIVFLGPPSSSMNALGDKVGSALIAQAAGVPTLPWSGSQVEIPLEVCLDSIPAEMYRKACVSTTEEALASCQMIGYPAMIKASWGGGGKGIRKVNNDDDVRALFKQVQGEVPGSPIFIMRLASQSRHLEVQLLCDQYGNVAALHSRDCSVQRRHQKIIEEGPVTVAPRETVKELEQAARRLAKAVGYVGAATVEYLYSMETGEYYFLELNPRLQVEHPVTEWIAEVNLPAAQVAVGMGIPLWQVPEIRRFYGMDNGGGYDIWRKTAALATPFNFDEVDSQWPKGHCVAVRITSEDPDDGFKPTGGKVKEISFKSKPNVWAYFSVKSGGGIHEFADSQFGHVFAYGVSRAAAITNMSLALKEIQIRGEIHSNVDYTVDLLNASDFKENRIHTGWLDNRIAMRVQAERPPWYISVVGGALYKTITSNTDTVSEYVSYLVKGQIPPKHISLVHSTVSLNIEESKYTIETIRSGQGSYRLRMNGSVIEANVQTLCDGGLLMQLDGNSHVIYAEEEAGGTRLLIDGKTCLLQNDHDPSRLLAETPCKLLRFLVADGAHVEADVPYAEVEVMKMCMPLLSPAAGVINVLLSEGQPMQAGDLIARLDLDDPSAVKRAEPFNGSFPEMSLPIAASGQVHKRCATSLNAARMVLAGYDHPINKVVQDLVSCLDAPELPFLQWEELMSVLATRLPRLLKSELEGKYSEYKLNVGHGKSKDFPSKMLREIIEENLAHGSEKEIATNERLVEPLMSLLKSYEGGRESHAHFIVKSLFEDYLSVEELFSDGIQSDVIERLRQQHSKDLQKVVDIVLSHQGVRNKTKLILTLMEKLVYPNPAVYKDQLTRFSSLNHKRYYKLALKASELLEQTKLSELRTSIARSLSELEMFTEERTAISEIMGDLVTAPLPVEDALVSLFDCSDQTLQQRVIETYISRLYQPHLVKDSIQLKYQESGVIALWEFAEAHSEKRLGAMVIVKSLESVSAAIGAALKGTSRYASSEGNIMHIALLGADNQMHGTEDSGDNDQAQVRIDKLSATLEQNTVTADLRAAGVKVISCIVQRDGALMPMRHTFLLSDEKLCYEEEPVLRHVEPPLSALLELGKLKVKGYNEVKYTPSRDRQWNIYTLRNTENPKMLHRVFFRTLVRQPGASNKFTSGNISDVEVGGAEESLSFTSSSILRSLMTAIEELELHAIRTGHSHMFLCILKEQKLLDLVPVSGNKVVDIGQDEATACLLLKEMALQIHELVGARMHHLSVCQWEVKLKLDSDGPASGTWRVVTTNVTSHTCTVDIYREVEDTESQKLVYHSAPSSSGPLHGVALNTPYQPLSVIDLKRCSARNNRTTYCYDFPLAFETAVQKSWSNISSDTNRCYVKATELVFAHKNGSWGTPVIPMERPAGLNDIGMVAWILDMSTPEYPNGRQIVVIANDITFRAGSFGPREDAFFETVTNLACERKLPLIYLAANSGARIGIADEVKSCFRVGWSDDGSPERGFQYIYLTEEDHARISASVIAHKMQLDNGEIRWVIDSVVGKEDGLGVENIHGSAAIASAYSRAYEETFTLTFVTGRTVGIGAYLARLGIRCIQRTDQPIILTGFSALNKLLGREVYSSHMQLGGPKIMATNGVVHLTVSDDLEGVSNILRWLSYVPANIGGPLPITKSLDPPDRPVAYIPENTCDPRAAISGIDDSQGKWLGGMFDKDSFVETFEGWAKSVVTGRAKLGGIPVGVIAVETQTMMQLIPADPGQLDSHERSVPRAGQVWFPDSATKTAQAMLDFNREGLPLFILANWRGFSGGQRDLFEGILQAGSTIVENLRTYNQPAFVYIPKAAELRGGAWVVIDSKINPDRIEFYAERTAKGNVLEPQGLIEIKFRSEELQECMGRLDPELINLKAKLQGVKHENGSLPESESLQKSIEARKKQLLPLYTQIAVRFAELHDTSLRMAAKGVIKKVVDWEDSRSFFYKRLRRRISEDVLAKEIRGVSGKQFSHQSAIELIQKWYLASKGAETGSTEWDDDDAFVAWRENPENYQEYIKELRAQRVSQLLSDVADSSPDLEALPQGLSMLLEKMDPSRRAQFVEEVKKVLK

SEQ ID NO: 17 - DNA, 6966 bp, Setaria italica
atgtcgcaacttggattagctgcagctgcctcaaaggcgctgccactacttcctaatcgccatagaacttcagctggaactacattcccatcacctgtatcatcgcggccctcaaaccgaaggaaaagccgcactcgttcacttcgtgatggaggagatggggtatcagatgccaaaaagcacaaccagtctgtccgtcaaggtcttgctggcatcatcgacctcccaaatgaggcaacatcggaagtggatatttctcatggatccgaggatcccagggggccaaccgattcatatcaaatgaatgggattgtaagtgaagcacataatggcagacatgcctcagtgtccaaggttgttgaattttgtgcggcgctaggtggcaaaacaccaattcacagtatactagtggccaacaatggaatggcagcagcaaagttcatgaggagtgtccggacatgggctaatgatacttttggatcggagaaggcgattcagctcatagctatggcaactccagaagacatgaggataaatgcagaacacattagaattgctgatcaatttgtggaggtgcctggtggaacaaacaataacaactatgcaaatgttcaactcatagtggaggtagcagaaagaataggtgtttctgctgtttggcctggttggggtcatgcttctgagaatcctgaacttccagatgcattgaccgcaaaaggagttgttttccttgggccacctgcggcatcaatgaatgcattgggagataaggtcggttcagctctcattgctcaagcagctggggtcccgaccctttcgtggagtggatcacatgttgaagttccattagagtgctgcttagatgcgatacctgaggaaatgtatagaaaagcttgtgttactaccacagaagaagctgttgcgagttgtcaggtggttggttatcctgccatgattaaggcatcctggggaggtggtggtaaaggaataagaaaggttcataatgacgatgaggttagagcactgtttaagcaagtacaaggtgaagtccctggctccccaatatttatcatgaggcttgcatcccagagtcgtcatcttgaagttcagttgctttgtgatcaatatggcaatgtggcagcacttcacagtcgtgattgcagtgtgcaacggcgacaccaaaagattattgaggaaggcccagttactgttgctcctcgtgagacagttaaagcgcttgagcaggcagcaaggaggcttgctaaggctgtgggttatgttggtgctgctactgttgaatacctttacagcatggagactggggaatactattttctggagcttaatcccagattacaggtcgagcatccagtcactgagtggattgctgaagtaaatcttcctgcagctcaagttgcagttggaatgggcatacctctttggcagattccagaaatcagacgtttcgatggaatggactatggaggaggatatgacatttggaggaaaacagcagctcttgccacaccatttaattttgatgaagtagattctcaatggccaaagggccattgtgtagcagttagaattactagcgaggatccagatgatggtttcaaacctactggtgggaaagtgaaggagataagttttaaaagcaagcctaatgtttgggcctacttctcagtaaagtctggtggaggcattcatgaatttgttgattctcagtttgggcatgtttttgcatatgggctctctagatcagcagcaataacgaacatggctcttgcattaaaagagattcaaattcgtggagaaattcattcaaatgttgattacacagttgatctcttaaatgcttcagacttcagagaaaataagattcatactggctggcttgataccagaatagctatgcgtgttcaagctgagaggcccccatggtatatttcagtggttggaggagctctatataaaacagtaactgccaatgcagccactgtttctgattatgtcagttatctcaccaagggccagattccaccaaagcatatatcccttgtcagttcaacagttaatctgaatatcgaagggagcaaatacacagttgaaactgtaaggactggacatggtagctacagattacgaatgaatgattcagcaattgaagcgaatgtacaatccttatgtgatggaggcctcttaatgcagttggatggaaatagccatgtaatttacgcggaagaagaagctggtggtacacgacttctgattgatggaaagacatgcttgttacagaatgatcatgatccatcaaagttattagctgagacaccctgcaaacttcttcggttcttggttgctgatggtgcccatgttgatgctgatgtaccatatgcggaagttgaggttatgaaaatgtgcatgcctctcttgtcgcctgcttctggtgtcattcatgttatgatgtctgagggccaggcattgcaggctggtgatcttatagcaaggctggatcttgatgacccttctgctgtgaaaagagctgaaccatttcatggaatatttccacaaatggaccttcctgttgctgcctctagccaagtacacaaaagatatgctgcaagttggaatgctgctcgaatggtccttgcaggatacgagcataatatcaatgaagttgtacaagatttggtatgctgcctggatgatcccgagcttcccttcctacagtgggatgaacttatgtcagttctagcaactaggcttccaagaaatcttaagagtgagttagaggataaatacatggaatacaagttgaacttttaccatgggaaaaacaaggacttcccgtccaagctgctgagagacatcattgaggcaaatcttgcatatggttcagagaaggaaaaagctacgaatgagaggcttattgagcctcttatgagcctacttaagtcatatgagggtgggagagaaagccatgctcattttgttgtcaagtcccttttcaaggagtaccttgctgtggaagaacttttcagtgatgggattcagtctgatgtgattgaaaccctgcgtcatcagcacagtaaagacttgcagaaggttgtagacattgtgttgtctcaccagggtgtgaggaacaaagctaagcttgtaacagcacttatggaaaagctggtttatccaaatcctgctgcttacagggatctgttggttcgcttttcttcactcaatcataaaagatattataagttggcccttaaagcaagcgaacttcttgaacaaactaaactaagtgaactccgtgcaagcatcgcaagaagcctttctgatctggggatgcataagggagaaatgactattgaagatagcatggaagatttagtctctgccccattacctgtcgaagatgcacttatttctttgtttgattacagtgatccaactgttcagcagaaagtgatcgagacatacatatctcgattgtatcagcctcttcttgtgaaagatagcatccaagtgaaatttaaggaatctggtgcctttgctttatgggaattttctgaagggcatgttgatactaaaaatggacaagggaccgttcttggtcgaacaagatggggtgccatggtagctgtcaaatcagttgaatctgcacgaacagccattgtagctgcattaaaggattcggcacagcatgccagctctgagggcaacatgatgcacattgccttattgagtgctgaaaatgaaaataatatcagtgatgatcaagctcaacataggatggaaaaacttaacaagatactcaaggatactagtgtcgcaaatgatcttcgagctgctggtttgaaggttataagttgcattgttcaaagagatgaagcacgcatgccaatgcgccacacattactctggtcagatgaaaagagttgttatgaggaagagcagattcttcggcatgtggagcctcccctctccatgcttcttgaaatggataagttgaaagtgaaaggatacaatgaaatgaagtatactccatcacgtgatcgtcaatggcatatctacacactaagaaatactgaaaaccccaaaatgttgcatagggtatttttccgaactattgtcaggcaacccaatgcaggcaacaagtttatatcagcccaaattggcgacactgaagtaggaggtcctgaggaatctttgtcatttacatctaatagcattttaagagccttgatgactgctattgaagaattagagcttcatgcaattaggactgatcattctcacatgtatttgtgcatattgaaagaacaaaagcttcttgatctcattccgttttcagggagcacaatcgtcgatgttgtccaagacgaagctactgcttgttcacttttaaaatcaatggctttgaagatacacgaacttgttggtgcacagatgcatcatctttctgtatgccagtgggaggtgaaactcaagttgtactgcgatgggcctgccagtggcacctggagagttgtaactacaaatgttactagtcacacttgcaccgttgatatctaccgggaagtggaagatactgaatcgcagaagttagtataccattcagcttctccgtcagctagtcctttgcatggtgtggccctggataatccgtatcaacctttgagtgtcattgatctaaaacactgctctgctaggaacaacagaactacatattgctatgattttccactggcatttgaaactgccctgcagaagtcatggcagtccaatggctccagtgtttctgaaggcagtgaaaatagtaggtcttatgtgaaagcaacagagctggtgtttgctgaaaaacatgggtcctggggcactcctataatttccatggagcgtcccgctgggctcaatgacattggcatggtagcttggatcttagagatgtccactcctgaatttcccaatggcaggcagattattgtcatagcaaatgatattactttcagagctggatcatttggcccaagggaagatgcgttttttgaagctgtcacgaacctggcctgcgagaggaagcttcctcttatatacttggcagcaaactccggtgctaggattggcatagccgatgaagtgaaatcttgcttccgtgttgggtggtccgatgaaggcagccctgaacggggttttcagtacatttatctgactgacgaagactatgcccgtattagcttgtctgttatagcacacaagctgcagctggataatggtgaaattaggtggattattgactctgttgtgggcaaggaggatgggcttggtgttgagaatatacatggaagtgctgctattgccagtgcttattctagggcatatgaggagacatttacacttacatttgtgactgggcggactgttggaataggagcatatcttgctcggctcggtatacggtgcatacagcgtcttgaccagcctattattttaactgggttttctgccctgaacaagcttcttgggcgggaagtgtacagctcccacatgcagttgggtggtcctaagatcatggcgaccaatggtgttgtccacttgactgtttcagatgaccttgaaggtgtttccaatatattgaggtggctcagctatgttcctgccaacattggtggacctcttcctattacaaaacctttggacccaccagacagacctgttgcatacatccctgagaacacatgtgatccgcgcgcagccattcgtggtgtagatgacagccaagggaaatggttgggtggtatgtttgacaaagacagctttgtcgagacatttgaaggatgggcgaaaacagtggttacgggcagagcaaagcttggaggaattcctgttggcgtcatagctgtggagacacaaaccatgatgcagcttatccctgctgatccaggccagcttgattcccatgagcgatctgttcctcgggctggacaagtgtggttcccagattctgcaaccaagacagctcaggcattgttggacttcaaccgtgaaggattgccgctgttcatccttgctaactggagaggattctctggtggacaaagagatctgtttgaaggaattcttcaggctgggtcaacaattgttgagaaccttaggacatacaatcagcctgcttttgtctacattcctatggctggagagctgcgtggaggagcttgggttgtggttgatagcaaaataaatccagaccgaattgagtgttatgctgagaggactgctaaaggcaatgttctggaacctcaagggttaattgaaatcaaattcagatcagaggagctccaagactgtatgggtaggcttgacccagggttgataaatctgaaagcaaaactccaaggtgcaaagcttggaaatggaagcctaacagatgtagaatcccttcagaagagtatagatgctcgtacgaaacagttgttgcctttatacacccagattgcaatacggtttgctgaattgcatgatacttccctcagaatggcagctaaaggtgtgattaagaaagttgtagattgggaagaatcacgttctttcttctacagaaggctacggaggaggatctctgaagatgttcttgcaaaagaaataagaggaatagctggtgaccacttcactcaccaatcagcagttgagctgatcaaggaatggtacttggcttctcaagccacaacaggaagcactgaatgggatgatgatgatgcttttgttgcctggaaggagaatcctgaaaactataagggatatatccaagagttaagggctcaaaaggtgtctcagtcgctctccgatcttgcagactccagttcagatctagaagcattctcacagggtctttccacattattagataagatggatccctctcagagagccaagttcattcaggaagtcaagaaggtcctgggttga

SEQ ID NO: 18 - protein, 2321 aa, Setaria italica
MSQLGLAAAASKALPLLPNRHRTSAGTTFPSPVSSRPSNRRKSRTRSLRDGGDGVSDAKKHNQSVRQGLAGIIDLPNEATSEVDISHGSEDPRGPTDSYQMNGIVSEAHNGRHASVSKVVEFCAALGGKTPIHSILVANNGMAAAKFMRSVRTWANDTFGSEKAIQLIAMATPEDMRINAEHIRIADQFVEVPGGTNNNNYANVQLIVEVAERIGVSAVWPGWGHASENPELPDALTAKGVVFLGPPAASMNALGDKVGSALIAQAAGVPTLSWSGSHVEVPLECCLDAIPEEMYRKACVTTTEEAVASCQVVGYPAMIKASWGGGGKGIRKVHNDDEVRALFKQVQGEVPGSPIFIMRLASQSRHLEVQLLCDQYGNVAALHSRDCSVQRRHQKIIEEGPVTVAPRETVKALEQAARRLAKAVGYVGAATVEYLYSMETGEYYFLELNPRLQVEHPVTEWIAEVNLPAAQVAVGMGIPLWQIPEIRRFDGMDYGGGYDIWRKTAALATPFNFDEVDSQWPKGHCVAVRITSEDPDDGFKPTGGKVKEISFKSKPNVWAYFSVKSGGGIHEFVDSQFGHVFAYGLSRSAAITNMALALKEIQIRGEIHSNVDYTVDLLNASDFRENKIHTGWLDTRIAMRVQAERPPWYISVVGGALYKTVTANAATVSDYVSYLTKGQIPPKHISLVSSTVNLNIEGSKYTVETVRTGHGSYRLRMNDSAIEANVQSLCDGGLLMQLDGNSHVIYAEEEAGGTRLLIDGKTCLLQNDHDPSKLLAETPCKLLRFLVADGAHVDADVPYAEVEVMKMCMPLLSPASGVIHVMMSEGQALQAGDLIARLDLDDPSAVKRAEPFHGIFPQMDLPVAASSQVHKRYAASWNAARMVLAGYEHNINEVVQDLVCCLDDPELPFLQWDELMSVLATRLPRNLKSELEDKYMEYKLNFYHGKNKDFPSKLLRDIIEANLAYGSEKEKATNERLIEPLMSLLKSYEGGRESHAHFVVKSLFKEYLAVEELFSDGIQSDVIETLRHQHSKDLQKVVDIVLSHQGVRNKAKLVTALMEKLVYPNPAAYRDLLVRFSSLNHKRYYKLALKASELLEQTKLSELRASIARSLSDLGMHKGEMTIEDSMEDLVSAPLPVEDALISLFDYSDPTVQQKVIETYISRLYQPLLVKDSIQVKFKESGAFALWEFSEGHVDTKNGQGTVLGRTRWGAMVAVKSVESARTAIVAALKDSAQHASSEGNMMHIALLSAENENNISDDQAQHRMEKLNKILKDTSVANDLRAAGLKVISCIVQRDEARMPMRHTLLWSDEKSCYEEEQILRHVEPPLSMLLEMDKLKVKGYNEMKYTPSRDRQWHIYTLRNTENPKMLHRVFFRTIVRQPNAGNKFISAQIGDTEVGGPEESLSFTSNSILRALMTAIEELELHAIRTDHSHMYLCILKEQKLLDLIPFSGSTIVDVVQDEATACSLLKSMALKIHELVGAQMHHLSVCQWEVKLKLYCDGPASGTWRVVTTNVTSHTCTVDIYREVEDTESQKLVYHSASPSASPLHGVALDNPYQPLSVIDLKHCSARNNRTTYCYDFPLAFETALQKSWQSNGSSVSEGSENSRSYVKATELVFAEKHGSWGTPIISMERPAGLNDIGMVAWILEMSTPEFPNGRQIIVIANDITFRAGSFGPREDAFFEAVTNLACERKLPLIYLAANSGARIGIADEVKSCFRVGWSDEGSPERGFQYIYLTDEDYARISLSVIAHKLQLDNGEIRWIIDSVVGKEDGLGVENIHGSAAIASAYSRAYEETFTLTFVTGRTVGIGAYLARLGIRCIQRLDQPIILTGFSALNKLLGREVYSSHMQLGGPKIMATNGVVHLTVSDDLEGVSNILRWLSYVPANIGGPLPITKPLDPPDRPVAYIPENTCDPRAAIRGVDDSQGKWLGGMFDKDSFVETFEGWAKTVVTGRAKLGGIPVGVIAVETQTMMQLIPADPGQLDSHERSVPRAGQVWFPDSATKTAQALLDFNREGLPLFILANWRGFSGGQRDLFEGILQAGSTIVENLRTYNQPAFVYIPMAGELRGGAWVVVDSKINPDRIECYAERTAKGNVLEPQGLIEIKFRSEELQDCMGRLDPGLINLKAKLQGAKLGNGSLTDVESLQKSIDARTKQLLPLYTQIAIRFAELHDTSLRMAAKGVIKKVVDWEESRSFFYRRLRRRISEDVLAKEIRGIAGDHFTHQSAVELIKEWYLASQATTGSTEWDDDDAFVAWKENPENYKGYIQELRAQKVSQSLSDLADSSSDLEAFSQGLSTLLDKMDPSQRAKFIQEVKKVLG

SEQ ID NO: 19 - DNA, 6966 bp, Setaria italica
atgtcgcaacttggattagctgcagctgcctcaaaggcgctgccactacttcctaatcgccatagaacttcagctggaactacattcccatcacctgtatcatcgcggccctcaaaccgaaggaaaagccgcactcgttcacttcgtgatggaggagatggggtatcagatgccaaaaagcacaaccagtctgtccgtcaaggtcttgctggcatcatcgacctcccaaatgaggcaacatcggaagtggatatttctcatggatccgaggatcccagggggccaaccgattcatatcaaatgaatgggattgtaaatgaagcacataatggcagacatgcctcagtgtccaaggttgttgaattttgtgcggcgctaggtggcaaaacaccaattcacagtatactagtggccaacaatggaatggcagcagcaaagttcatgaggagtgtccggacatgggctaatgatacttttggatcggagaaggcgattcagctcatagctatggcaactccagaagacatgaggataaatgcagaacacattagaattgctgatcaatttgtagaggtgcctggtggaacaaacaataacaactatgcaaatgttcaactcatagtggaggtagcagaaagaataggtgtttctgctgtttggcctggttggggtcatgcttctgagaatcctgaacttccagatgcattgaccgcaaaaggaattgttttccttgggccacctgcggcatcaatgaatgcattgggagataaggtcggttcagctctcattgctcaagcagctggggtcccgaccctttcgtggagtggatcacatgttgaagttccattagagtgctgcttagatgcgatacctgaggaaatgtatagaaaagcttgtgttactaccacagaagaagctgttgcgagttgtcaggtggttggttatcctgccatgattaaggcatcctggggaggtggtggtaaaggaataagaaaggttcataatgacgatgaggttagagcactgtttaagcaagtacaaggtgaagtccctggctccccaatatttatcatgaggcttgcatcccagagtcgtcatcttgaagttcagttgctttgtgatcaatatggcaatgtggcagcacttcacagtcgtgattgcagtgtgcaacggcgacaccaaaagattattgaggaaggcccagttactgttgctcctcgtgagacagttaaagcgcttgagcaggcagcaaggaggcttgctaaggctgtgggttatgttggtgctgctactgttgaatacctttacagcatggagactggggaatactattttctggagcttaatcccagattacaggtcgagcatccagtcactgagtggattgctgaagtaaatcttcctgcagctcaagttgcagttggaatgggcatacctctttggcagattccagaaatcagacgtttctatggaatggactatggaggaggatatgacatttggaggaaaacagcagctcttgccacaccatttaattttgatgaagtagattctcaatggccaaagggccattgtgtagcagttagaattactagcgaggatccagatgatggtttcaaacctactggtgggaaagtgaaggagataagttttaaaagcaagcctaatgtttgggcctacttctcagtaaagtctggtggaggcattcatgaatttgctgattctcagtttgggcatgtttttgcatatgggctctctagatcagcagcaataacgaacatggctcttgcattaaaagagattcaaattcgtggagaaattcattcaaatgttgattacacagttgatctcttaaatgcttcagacttcagagaaaataagattcatactggctggcttgataccagaatagctatgcgtgttcaagctgagaggcccccatggtatatttcagtggttggaggagctctatataaaacagtaactgccaatgcagccactgtttctgattatgtcagttatctcaccaagggccagattccaccaaagcatatatcccttgtcagttcaacagttaatctgaatatcgaagggagcaaatacacagttgaaactgtaaggactggacatggtagctacagattacgaatgaatgattcagcaattgaagcgaatgtacaatctttatgtgatggaggcctcttaatgcagttggatggaaatagccatgtaatttacgcggaagaagaagctggtggtacacgacttctgattgatggaaagacatgcttgttacagaatgatcatgatccatcaaagttattagctgagacaccctgcaaacttcttcggttcttggttgctgatggtgctcatgttgatgctgatgtaccatatgcggaagttgaggttatgaaaatgtgcatgcctctcttgtcgcctgcttctggtgtcattcatgttatgatgtctgagggccaggcattgcaggctggtgatcttatagcaaggctggatcttgatgacccttctgctgtgaaaagagctgaaccatttcatggaatatttccacaaatggaccttcctgttgctgcctctagccaagtacacaaaagatatgctgcaagtttgaatgctgctcgaatggtccttgcaggatacgagcataatatcaatgaagttgtacaagatttggtatgctgcctggatgatcccgagcttcccttcctacagtgggatgaacttatgtcagttctagcaactaggcttccaagaaatcttaagagtgagttagaggataaatacatggaatacaagttgaacttttaccatgggaaaaacaaggacttcccgtccaagctgctgagagacatcattgaggcaaatcttgcatatggttcagagaaggaaaaagctacgaatgagaggcttattgagcctcttatgagcctacttaagtcatatgagggtgggagagaaagccatgctcattttgttgtcaagtcccttttcaaggagtaccttgctgtggaagaacttttcagtgatgggattcagtctgatgtgattgaaaccctgcgtcatcagcacagtaaagacttgcagaaggttgtagacattgtgttgtctcaccagggtgtgaggaacaaagctaagcttgtaacagcacttatggaaaagctggtttatccaaatcctgctgcttacagggatctgttggttcgcttttcttcactcaatcataaaagatattataagttggcccttaaagcaagcgaacttcttgaacaaactaaactaagtgaactccgtgcaagcatcgcaagaagcctttctgatctggggatgcataagggagaaatgactattgaagatagcatggaagatttagtctctgccccattacctgtcgaagatgcacttatttctttgtttgattacagtgatccaactgttcagcagaaagtgatcgagacatacatatctcgattgtatcagcctcttcttgtgaaagatagcatccaagtgaaatttaaggaatctggtgcctttgctttatgggaattttctgaagggcatgttgatactaaaaatggacaagggaccgttcttggtcgaacaagatggggtgccatggtagctgtcaaatcagttgaatctgcacgaacagccattgtagctgcattaaaggattcggcacagcatgccagctctgagggcaacatgatgcacattgccttattgagtgctgaaaatgaaaataatatcagtgatgatcaagctcaacataggatggaaaaacttaacaagatactcaaggatactagtgtcgcaaatgatcttcgagctgctggtttgaaggttataagttgcattgttcaaagagatgaagcacgcatgccaatgcgccacacattactctggtcagatgaaaagagttgttatgaggaagagcagattcttcggcatgtggagcctcccctctccatgcttcttgaaatggataagttgaaagtgaaaggatacaatgaaatgaagtatactccatcacgtgatcgtcaatggcatatctacacactaagaaatactgaaaaccccaaaatgttgcatagggtatttttccgaactattgtcaggcaacccaatgcaggcaacaagtttatatcagcccaaattggcgacactgaagtaggaggtcctgaggaatctttgtcatttacatctaatagcattttaagagccttgatgactgctattgaagaattagagcttcatgcaattaggactggtcattctcacatgtatttgtgcatattgaaagaacaaaagcttcttgatctcattccgttttcagggagcacaatcgtcgatgttggccaagacgaagctactgcttgttcacttttaaaatcaatggctttgaagatacacgaacttgttggtgcacagatgcatcatctttctgtatgccagtgggaggtgaaactcaagttgtactgcgatgggcctgccagtggcacctggagagttgtaactacaaatgttactagtcacacttgcaccattgatatctaccgggaagtggaagatactgaatcgcagaagttagtataccattcagcttctccgtcagctagtcctttgcatggtgtggccctggataatccgtatcaacctttgagtgtcattgatctaaaacgctgctctgctaggaacaacagaactacatattgctatgattttccactggcatttgaaactgccctgcagaagtcatggcagtccaatggctccagtgtttctgaaggcagtgaaaatagtaggtcttatgtgaaagcaacagagctggtgtttgctgaaaaacatgggtcctggggcactcctataatttccatggagcgtcccgctgggctcaatgacattggcatggtagcttggatcttagagatgtccactcctgaatttcccaatggcaggcagattattgtcatagcaaatgatattactttcagagctggatcatttggcccaagggaagatgcgttttttgaagctgtcacgaacctggcctgcgagaggaagcttcctcttatatacttggcagcaaactccggtgctaggattggcatagccgatgaagtgaaatcttgcttccgtgttgggtggtccgatgaaggcagccctgaacggggttttcagtacatttatctgactgacgaagactatgcccgtattagcttgtctgttatagcacacaagctgcagctggataatggtgaaattaggtggattattgactctgttgtgggcaaggaggatgggcttggtgttgagaatctacatggaagtgctgctattgccagtgcttattctagggcatatgaggagacatttacacttacatttgtgactgggcggactgttggaataggagcatatctcgctcggctcggtatacggtgcatacagcgtcttgaccagcctattattttaactgggttttctgccctgaacaagcttcttgggcgggaagtgtacagctcccacatgcagttgggtggtcctaagatcatggcgaccaatggtgttgtccacttgactgtttcagatgaccttgaaggtgtttccaatatattgaggtggctcagctatgttcctgccaacattggtggacctcttcctattacaaaacctttggacccaccagacagacctgttgcatacatccctgagaacacatgtgatccgcgcgcagccattcgtggtgtagatgacagccaagggaaatggttgggtggtatgtttgacaaagacagctttgtcgagacatttgaaggatgggcgaaaacagtggttacgggcagagcaaagcttggaggaattcctgttggtgtcatagctgtggagacacaaaccatgatgcagcttatccctgctgatccaggccagcttgattcccatgagcgatctgttcctcgggctggacaagtgtggttcccagattctgcaaccaagacagctcaggcattgttggacttcaaccgtgaaggattgccgctgttcatccttgctaactggagaggattctctggtggacaaagagatctgtttgaaggaattcttcaggctgggtcaacaattgttgagaaccttaggacatacaatcagcctgcttttgtctacattcctatggctggagagctgcgtggaggagcttgggttgtggttgatagcaaaataaatccagaccgaattgagtgttatgctgagaggactgctaaaggcaatgttcttgaacctcaagggttaattgaaatcaaattcagatcagaggagctccaagactgtatgggtaggcttgacccagagttgataaatctgaaagcaaaactccaaggtgcaaagcttggaaatggaagcctaacagatgtagaatcccttcagaagagtatagatgctcgtacgaaacagttgttgcctttatacacccagattgcaatacggtttgctgaattgcatgatacttccctcagaatggcagctaaaggtgtgattaagaaagttgtagattgggaagaatcacgttctttcttctacagaaggctacggaggaggatctctgaagatgttcttgcaaaagaaataagaggaatagctggtgaccacttcactcaccaatcagcagttgagctgatcaaggaatggtacttggcttctcaagccacaacaggaagcactgaatgggatgatgatgatgcttttgttgcctggaaggagaatcctgaaaactataagggatatatccaagagttaagggctcaaaaggtgtctcagtcgctctccgatcttgcagactccagttcagatctagaagcattctcacagggtctttccacattattagataagatggatccctctcagagagccaagttcattcaggaagtcaagaaggtcctgggttga

SEQ ID NO: 20 - protein, 2321 aa, Setaria italica
MSQLGLAAAASKALPLLPNRHRTSAGTTFPSPVSSRPSNRRKSRTRSLRDGGDGVSDAKKHNQSVRQGLAGIIDLPNEATSEVDISHGSEDPRGPTDSYQMNGIVNEAHNGRHASVSKVVEFCAALGGKTPIHSILVANNGMAAAKFMRSVRTWANDTFGSEKAIQLIAMATPEDMRINAEHIRIADQFVEVPGGTNNNNYANVQLIVEVAERIGVSAVWPGWGHASENPELPDALTAKGIVFLGPPAASMNALGDKVGSALIAQAAGVPTLSWSGSHVEVPLECCLDAIPEEMYRKACVTTTEEAVASCQVVGYPAMIKASWGGGGKGIRKVHNDDEVRALFKQVQGEVPGSPIFIMRLASQSRHLEVQLLCDQYGNVAALHSRDCSVQRRHQKIIEEGPVTVAPRETVKALEQAARRLAKAVGYVGAATVEYLYSMETGEYYFLELNPRLQVEHPVTEWIAEVNLPAAQVAVGMGIPLWQIPEIRRFYGMDYGGGYDIWRKTAALATPFNFDEVDSQWPKGHCVAVRITSEDPDDGFKPTGGKVKEISFKSKPNVWAYFSVKSGGGIHEFADSQFGHVFAYGLSRSAAITNMALALKEIQIRGEIHSNVDYTVDLLNASDFRENKIHTGWLDTRIAMRVQAERPPWYISVVGGALYKTVTANAATVSDYVSYLTKGQIPPKHISLVSSTVNLNIEGSKYTVETVRTGHGSYRLRMNDSAIEANVQSLCDGGLLMQLDGNSHVIYAEEEAGGTRLLIDGKTCLLQNDHDPSKLLAETPCKLLRFLVADGAHVDADVPYAEVEVMKMCMPLLSPASGVIHVMMSEGQALQAGDLIARLDLDDPSAVKRAEPFHGIFPQMDLPVAASSQVHKRYAASLNAARMVLAGYEHNINEVVQDLVCCLDDPELPFLQWDELMSVLATRLPRNLKSELEDKYMEYKLNFYHGKNKDFPSKLLRDIIEANLAYGSEKEKATNERLIEPLMSLLKSYEGGRESHAHFVVKSLFKEYLAVEELFSDGIQSDVIETLRHQHSKDLQKVVDIVLSHQGVRNKAKLVTALMEKLVYPNPAAYRDLLVRFSSLNHKRYYKLALKASELLEQTKLSELRASIARSLSDLGMHKGEMTIEDSMEDLVSAPLPVEDALISLFDYSDPTVQQKVIETYISRLYQPLLVKDSIQVKFKESGAFALWEFSEGHVDTKNGQGTVLGRTRWGAMVAVKSVESARTAIVAALKDSAQHASSEGNMMHIALLSAENENNISDDQAQHRMEKLNKILKDTSVANDLRAAGLKVISCIVQRDEARMPMRHTLLWSDEKSCYEEEQILRHVEPPLSMLLEMDKLKVKGYNEMKYTPSRDRQWHIYTLRNTENPKMLHRVFFRTIVRQPNAGNKFISAQIGDTEVGGPEESLSFTSNSILRALMTAIEELELHAIRTGHSHMYLCILKEQKLLDLIPFSGSTIVDVGQDEATACSLLKSMALKIHELVGAQMHHLSVCQWEVKLKLYCDGPASGTWRVVTTNVTSHTCTIDIYREVEDTESQKLVYHSASPSASPLHGVALDNPYQPLSVIDLKRCSARNNRTTYCYDFPLAFETALQKSWQSNGSSVSEGSENSRSYVKATELVFAEKHGSWGTPIISMERPAGLNDIGMVAWILEMSTPEFPNGRQIIVIANDITFRAGSFGPREDAFFEAVTNLACERKLPLIYLAANSGARIGIADEVKSCFRVGWSDEGSPERGFQYIYLTDEDYARISLSVIAHKLQLDNGEIRWIIDSVVGKEDGLGVENLHGSAAIASAYSRAYEETFTLTFVTGRTVGIGAYLARLGIRCIQRLDQPIILTGFSALNKLLGREVYSSHMQLGGPKIMATNGVVHLTVSDDLEGVSNILRWLSYVPANIGGPLPITKPLDPPDRPVAYIPENTCDPRAAIRGVDDSQGKWLGGMFDKDSFVETFEGWAKTVVTGRAKLGGIPVGVIAVETQTMMQLIPADPGQLDSHERSVPRAGQVWFPDSATKTAQALLDFNREGLPLFILANWRGFSGGQRDLFEGILQAGSTIVENLRTYNQPAFVYIPMAGELRGGAWVVVDSKINPDRIECYAERTAKGNVLEPQGLIEIKFRSEELQDCMGRLDPELINLKAKLQGAKLGNGSLTDVESLQKSIDARTKQLLPLYTQIAIRFAELHDTSLRMAAKGVIKKVVDWEESRSFFYRRLRRRISEDVLAKEIRGIAGDHFTHQSAVELIKEWYLASQATTGSTEWDDDDAFVAWKENPENYKGYIQELRAQKVSQSLSDLADSSSDLEAFSQGLSTLLDKMDPSQRAKFIQEVKKVLG

SEQ ID NO: 21 - DNA, 6966 bp, Setaria italica
atgtcgcaacttggattagctgcagctgcctcaaaggcgctgccactacttcctaatcgccatagaacttcagctggaactacattcccatcacctgtatcatcgcggccctcaaaccgaaggaaaagccgcactcgttcacttcgtgatggaggagatggggtatcagatgccaaaaagcacaaccagtctgtccgtcaaggtcttgctggcatcatcgacctcccaaatgaggcaacatcggaagtggatatttctcatggatccgaggatcccagggggccaaccgattcatatcaaatgaatgggattgtaaatgaagcacataatggcagacatgcctcagtgtccaaggttgttgaattttgtgcggcgctaggtggcaaaacaccaattcacagtatactagtggccaacaatggaatggcagcagcaaagttcatgaggagtgtccggacatgggctaatgatacttttggatcggagaaggcgattcagctcatagctatggcaactccagaagacatgaggataaatgcagaacacattagaattgctgatcaatttgtagaggtgcctggtggaacaaacaataacaactatgcaaatgttcaactcatagtggaggtagcagaaagaataggtgtttctgctgtttggcctggttggggtcatgcttctgagaatcctgaacttccagatgcattgaccgcaaaaggaattgttttccttgggccacctgcggcatcaatgaatgcattgggagataaggtcggttcagctctcattgctcaagcagctggggtcccgaccctttcgtggagtggatcacatgttgaagttccattagagtgctgcttagatgcgatacctgaggaaatgtatagaaaagcttgtgttactaccacagaagaagctgttgcgagttgtcaggtggttggttatcctgccatgattaaggcatcctggggaggtggtggtaaaggaataagaaaggttcataatgacgatgaggttagagcactgtttaagcaagtacaaggtgaagtccctggctccccaatatttatcatgaggcttgcatcccagagtcgtcatcttgaagttcagttgctttgtgatcaatatggcaatgtggcagcacttcacagtcgtgattgcagtgtgcaacggcgacaccaaaagattattgaggaaggcccagttactgttgctcctcgtgagacagttaaagcgcttgagcaggcagcaaggaggcttgctaaggctgtgggttatgttggtgctgctactgttgaatacctttacagcatggagactggggaatactattttctggagcttaatcccagattacaggtcgagcatccagtcactgagtggattgctgaagtaaatcttcctgcagctcaagttgcagttggaatgggcatacctctttggcagattccagaaatcagacgtttctatggaatggactatggaggaggatatgacatttggaggaaaacagcagctcttgccacaccatttaattttgatgaagtagattctcaatggccaaagggccattgtgtagcagttagaattactagcgaggatccagatgatggtttcaaacctactggtgggaaagtgaaggagataagttttaaaagcaagcctaatgtttgggcctacttctcagtaaagtctggtggaggcattcatgaatttgctgattctcagtttgggcatgtttttgcatatgggctctctagatcagcagcaataacgaacatggctcttgcattaaaagagattcaaattcgtggagaaattcattcaaatgttgattacacagttgatctcttaaatgcttcagacttcagagaaaataagattcatactggctggcttgataccagaatagctatgcgtgttcaagctgagaggcccccatggtatatttcagtggttggaggagctctatataaaacagtaactgccaatgcagccactgtttctgattatgtcagttatctcaccaagggccagattccaccaaagcatatatcccttgtcagttcaacagttaatctgaatatcgaagggagcaaatacacagttgaaactgtaaggactggacatggtagctacagattacgaatgaatgattcagcaattgaagcgaatgtacaatctttatgtgatggaggcctcttaatgcagttggatggaaatagccatgtaatttacgcggaagaagaagctggtggtacacgacttctgattgatggaaagacatgcttgttacagaatgatcatgatccatcaaagttattagctgagacaccctgcaaacttcttcggttcttggttgctgatggtgctcatgttgatgctgatgtaccatatgcggaagttgaggttatgaaaatgtgcatgcctctcttgtcgcctgcttctggtgtcattcatgttatgatgtctgagggccaggcattgcaggctggtgatcttatagcaaggctggatcttgatgacccttctgctgtgaaaagagctgaaccatttcatggaatatttccacaaatggaccttcctgttgctgcctctagccaagtacacaaaagatatgctgcaagtttgaatgctgctcgaatggtccttgcaggatacgagcataatatcaatgaagttgtacaagatttggtatgctgcctggatgatcccgagcttcccttcctacagtgggatgaacttatgtcagttctagcaactaggcttccaagaaatcttaagagtgagttagaggataaatacatggaatacaagttgaacttttaccatgggaaaaacaaggacttcccgtccaagctgctgagagacatcattgaggcaaatcttgcatatggttcagagaaggaaaaagctacgaatgagaggcttattgagcctcttatgagcctacttaagtcatatgagggtgggagagaaagccatgctcattttgttgtcaagtcccttttcaaggagtaccttgctgtggaagaacttttcagtgatgggattcagtctgatgtgattgaaaccctgcgtcatcagcacagtaaagacttgcagaaggttgtagacattgtgttgtctcaccagggtgtgaggaacaaagctaagcttgtaacagcacttatggaaaagctggtttatccaaatcctgctgcttacagggatctgttggttcgcttttcttcactcaatcataaaagatattataagttggcccttaaagcaagcgaacttcttgaacaaactaaactaagtgaactccgtgcaagcatcgcaagaagcctttctgatctggggatgcataagggagaaatgactattgaagatagcatggaagatttagtctctgccccattacctgtcgaagatgcacttatttctttgtttgattacagtgatccaactgttcagcagaaagtgatcgagacatacatatctcgattgtatcagcctcttcttgtgaaagatagcatccaagtgaaatttaaggaatctggtgcctttgctttatgggaattttctgaagggcatgttgatactaaaaatggacaagggaccgttcttggtcgaacaagatggggtgccatggtagctgtcaaatcagttgaatctgcacgaacagccattgtagctgcattaaaggattcggcacagcatgccagctctgagggcaacatgatgcacattgccttattgagtgctgaaaatgaaaataatatcagtgatgatcaagctcaacataggatggaaaaacttaacaagatactcaaggatactagtgtcgcaaatgatcttcgagctgctggtttgaaggttataagttgcattgttcaaagagatgaagcacgcatgccaatgcgccacacattactctggtcagatgaaaagagttgttatgaggaagagcagattcttcggcatgtggagcctcccctctccatgcttcttgaaatggataagttgaaagtgaaaggatacaatgaaatgaagtatactccatcacgtgatcgtcaatggcatatctacacactaagaaatactgaaaaccccaaaatgttgcatagggtatttttccgaactattgtcaggcaacccaatgcaggcaacaagtttatatcagcccaaattggcgacactgaagtaggaggtcctgaggaatctttgtcatttacatctaatagcattttaagagccttgatgactgctattgaagaattagagcttcatgcaattaggactggtcattctcacatgtatttgtgcatattgaaagaacaaaagcttcttgatctcattccgttttcagggagcacaatcgtcgatgttggccaagacgaagctactgcttgttcacttttaaaatcaatggctttgaagatacacgaacttgttggtgcacagatgcatcatctttctgtatgccagtgggaggtgaaactcaagttgtactgcgatgggcctgccagtggcacctggagagttgtaactacaaatgttactagtcacacttgcaccgttgatatctaccgggaagtggaagatactgaatcgcagaagttagtataccattcagcttctccgtcagctagtcctttgcatggtgtggccctggataatccgtatcaacctttgagtgtcattgatctaaaacgctgctctgctaggaacaacagaactacatattgctatgattttccactggcatttgaaactgccctgcagaagtcatggcagtccaatggctccagtgtttctgaaggcagtgaaaatagtaggtcttatgtgaaagcaacagagctggtgtttgctgaaaaacatgggtcctggggcactcctataatttccatggagcgtcccgctgggctcaatgacattggcatggtagcttggatcttagagatgtccactcctgaatttcccaatggcaggcagattattgtcatagcaaatgatattactttcagagctggatcatttggcccaagggaagatgcgttttttgaagctgtcacgaacctggcctgcgagaggaagcttcctcttatatacttggcagcaaactccggtgctaggattggcatagccgatgaagtgaaatcttgcttccgtgttgggtggtccgatgaaggcagccctgaacggggttttcagtacatttatctgactgacgaagactatgcccgtattagcttgtctgttatagcacacaagctgcagctggataatggtgaaattaggtggattattgactctgttgtgggcaaggaggatgggcttggtgttgagaatatacatggaagtgctgctattgccagtgcttattctagggcatatgaggagacatttacacttacatttgtgactgggcggactgttggaataggagcatatcttgctcggctcggtatacggtgcatacagcgtcttgaccagcctattattttaactgggttttctgccctgaacaagcttcttgggcgggaagtgtacagctcccacatgcagttgggtggtcctaagatcatggcgaccaatggtgttgtccacttgactgtttcagatgaccttgaaggtgtttccaatatattgaggtggctcagctatgttcctgccaacattggtggacctcttcctattacaaaacctttggacccaccagacagacctgttgcatacatccctgagaacacatgtgatccgcgcgcagccattcgtggtgtagatgacagccaagggaaatggttgggtggtatgtttgacaaagacagctttgtcgagacatttgaaggatgggcgaaaacagtggttacgggcagagcaaagcttggaggaattcctgttggtgtcatagctgtggagacacaaaccatgatgcagcttatccctgctgatccaggccagcttgattcccatgagcgatctgttcctcgggctggacaagtgtggttcccagattctgcaaccaagacagctcaggcattgttggacttcaaccgtgaaggattgccgctgttcatccttgctaactggagaggattctctggtggacaaagagatctgtttgaaggaattcttcaggctgggtcaacaattgttgagaaccttaggacatacaatcagcctgcttttgtctacattcctatggctggagagctgcgtggaggagcttgggttgtggttgatagcaaaataaatccagaccgaattgagtgttatgctgagaggactgctaaaggcaatgttctggaacctcaagggttaattgaaatcaaattcagatcagaggagctccaagactgtatgggtaggcttgacccagagttgataaatctgaaagcaaaactccaaggtgcaaagcttggaaatggaagcctaacagatgtagaatcccttcagaagagtatagatgctcgtacgaaacagttgttgcctttatacacccagattgcaatacggtttgctgaattgcatgatacttccctcagaatggcagctaaaggtgtgattaagaaagttgtagattgggaagaattacgttctttcttctacagaaggctacggaggaggatctctgaagatgttcttgcaaaagaaataagaggaatagctggtgaccacttcactcaccaatcagcagttgagctgatcaaggaatggtacttggcttctcaagccacaacaggaagcactgaatgggatgatgatgatgcttttgttgcctggaaggagaatcctgaaaactataagggatatatccaagagttaagggctcaaaaggtgtctcagtcgctctccgatcttgcagactccagttcagatctagaagcattctcacagggtctttccacattattagataagatggatccctctcagagagccaagttcattcaggaagtcaagaaggtcctgggttga

SEQ ID NO: 22 - protein, 2321 aa, Setaria italica
MSQLGLAAAASKALPLLPNRHRTSAGTTFPSPVSSRPSNRRKSRTRSLRDGGDGVSDAKKHNQSVRQGLAGIIDLPNEATSEVDISHGSEDPRGPTDSYQMNGIVNEAHNGRHASVSKVVEFCAALGGKTPIHSILVANNGMAAAKFMRSVRTWANDTFGSEKAIQLIAMATPEDMRINAEHIRIADQFVEVPGGTNNNNYANVQLIVEVAERIGVSAVWPGWGHASENPELPDALTAKGIVFLGPPAASMNALGDKVGSALIAQAAGVPTLSWSGSHVEVPLECCLDAIPEEMYRKACVTTTEEAVASCQVVGYPAMIKASWGGGGKGIRKVHNDDEVRALFKQVQGEVPGSPIFIMRLASQSRHLEVQLLCDQYGNVAALHSRDCSVQRRHQKIIEEGPVTVAPRETVKALEQAARRLAKAVGYVGAATVEYLYSMETGEYYFLELNPRLQVEHPVTEWIAEVNLPAAQVAVGMGIPLWQIPEIRRFYGMDYGGGYDIWRKTAALATPFNFDEVDSQWPKGHCVAVRITSEDPDDGFKPTGGKVKEISFKSKPNVWAYFSVKSGGGIHEFADSQFGHVFAYGLSRSAAITNMALALKEIQIRGEIHSNVDYTVDLLNASDFRENKIHTGWLDTRIAMRVQAERPPWYISVVGGALYKTVTANAATVSDYVSYLTKGQIPPKHISLVSSTVNLNIEGSKYTVETVRTGHGSYRLRMNDSAIEANVQSLCDGGLLMQLDGNSHVIYAEEEAGGTRLLIDGKTCLLQNDHDPSKLLAETPCKLLRFLVADGAHVDADVPYAEVEVMKMCMPLLSPASGVIHVMMSEGQALQAGDLIARLDLDDPSAVKRAEPFHGIFPQMDLPVAASSQVHKRYAASLNAARMVLAGYEHNINEVVQDLVCCLDDPELPFLQWDELMSVLATRLPRNLKSELEDKYMEYKLNFYHGKNKDFPSKLLRDIIEANLAYGSEKEKATNERLIEPLMSLLKSYEGGRESHAHFVVKSLFKEYLAVEELFSDGIQSDVIETLRHQHSKDLQKVVDIVLSHQGVRNKAKLVTALMEKLVYPNPAAYRDLLVRFSSLNHKRYYKLALKASELLEQTKLSELRASIARSLSDLGMHKGEMTIEDSMEDLVSAPLPVEDALISLFDYSDPTVQQKVIETYISRLYQPLLVKDSIQVKFKESGAFALWEFSEGHVDTKNGQGTVLGRTRWGAMVAVKSVESARTAIVAALKDSAQHASSEGNMMHIALLSAENENNISDDQAQHRMEKLNKILKDTSVANDLRAAGLKVISCIVQRDEARMPMRHTLLWSDEKSCYEEEQILRHVEPPLSMLLEMDKLKVKGYNEMKYTPSRDRQWHIYTLRNTENPKMLHRVFFRTIVRQPNAGNKFISAQIGDTEVGGPEESLSFTSNSILRALMTAIEELELHAIRTGHSHMYLCILKEQKLLDLIPFSGSTIVDVGQDEATACSLLKSMALKIHELVGAQMHHLSVCQWEVKLKLYCDGPASGTWRVVTTNVTSHTCTVDIYREVEDTESQKLVYHSASPSASPLHGVALDNPYQPLSVIDLKRCSARNNRTTYCYDFPLAFETALQKSWQSNGSSVSEGSENSRSYVKATELVFAEKHGSWGTPIISMERPAGLNDIGMVAWILEMSTPEFPNGRQIIVIANDITFRAGSFGPREDAFFEAVTNLACERKLPLIYLAANSGARIGIADEVKSCFRVGWSDEGSPERGFQYIYLTDEDYARISLSVIAHKLQLDNGEIRWIIDSVVGKEDGLGVENIHGSAAIASAYSRAYEETFTLTFVTGRTVGIGAYLARLGIRCIQRLDQPIILTGFSALNKLLGREVYSSHMQLGGPKIMATNGVVHLTVSDDLEGVSNILRWLSYVPANIGGPLPITKPLDPPDRPVAYIPENTCDPRAAIRGVDDSQGKWLGGMFDKDSFVETFEGWAKTVVTGRAKLGGIPVGVIAVETQTMMQLIPADPGQLDSHERSVPRAGQVWFPDSATKTAQALLDFNREGLPLFILANWRGFSGGQRDLFEGILQAGSTIVENLRTYNQPAFVYIPMAGELRGGAWVVVDSKINPDRIECYAERTAKGNVLEPQGLIEIKFRSEELQDCMGRLDPELINLKAKLQGAKLGNGSLTDVESLQKSIDARTKQLLPLYTQIAIRFAELHDTSLRMAAKGVIKKVVDWEELRSFFYRRLRRRISEDVLAKEIRGIAGDHFTHQSAVELIKEWYLASQATTGSTEWDDDDAFVAWKENPENYKGYIQELRAQKVSQSLSDLADSSSDLEAFSQGLSTLLDKMDPSQRAKFIQEVKKVLG

SEQ ID NO: 23 - DNA, 6963 bp, Alopecurus myosuroides; identical to SEQ ID NO: 4

SEQ ID NO: 24 - protein, 2320 aa, Alopecurus myosuroides; identical to SEQ ID NO: 1

SEQ ID NO: 25 - DNA, 6936 bp, Aegilops tauschii
atgggatccacacatttgcccattgtcggccttaatgcctcgacaacaccatcgctatccactattcgcccggtaaattcagccggtgctgcattccaaccatctgccccttctagaacctccaagaagaaaagtcgtcgtgttcagtcattaagggatggaggcgatggaggcgtgtcagaccctaaccagtctattcgccaaggtcttgccggcatcattgacctcccaaaggagggcacatcagctccggaagtggatatttcacatgggtccgaagaacccaggggctcctaccaaatgaatgggatactgaatgaagcacataatgggaggcatgcttcgctgtctaaggttgtcgaattttgtatggcattgggcggcaaaacaccaattcatagtgtattagttgcgaacaatggaatggcagcagctaagttcatgcggagtgtccgaacatgggctaatgaaacatttgggtcagagaaggcaattcagttgatagctatggctactccagaagacatgaggataaatgcagagcacattagaattgctgatcaatttgttgaagtacccggtggaacaaacaataacaactatgcaaatgtccaactcatagtggagatagcagtgagaaccggtgtttctgctgtttggcctggttggggccatgcatctgagaatcctgaacttccagatgcactaaatgcaaacggaattgtttttcttgggccaccatcatcatcaatgaacgcactaggtgacaaggttggttcagctctcattgctcaagcagcaggggttccgactcttccttggagtggatcacaggtggaaattccattagaagtttgtttggactcgatacctgcggatatgtataggaaagcttgtgttagtactacggaggaagcacttgcgagttgtcagatgattgggtatccagccatgattaaagcatcatggggtggtggtggtaaagggatccgaaaggttaataacgacgatgatgtcagagcactgtttaagcaagtgcaaggtgaagttcctggctccccaatatttatcatgagacttgcatctcagagtcgacatcttgaagttcagttgctttgtgatcaatatggcaatgtagctgcgcttcacagtcgtgactgcagtgtgcaacggcgacaccaaaagattattgaggaaggaccagttactgttgctcctcgcgagacagtgaaagagctagagcaagcagcaaggaggcttgctaaggctgtgggttatgttggtgctgctactgttgaatatctctacagcatggagactggtgaatactattttctggaacttaatccacggttgcaggttgagcatccagtcaccgagtggatagctgaagtaaacttgcctgcagctcaagttgcagttggaatgggtatacccctttggcaggttccagagatcagacgtttctatggaatggacaatggaggaggctatgacatttggaggaaaacagcagctcttgctaccccatttaactttgatgaagtggattctcaatggccaaagggtcattgtgtagcagttaggataaccagtgaggatccagatgacggattcaagcctaccggtggaaaagtaaaggagatcagttttaaaagcaagccaaatgtttgggcctatttctctgttaagtccggtggaggcattcatgaatttgctgattctcagtttggacatgtttttgcatatggagtgtctagagcagcagcaataaccaacatgtctcttgcgctaaaagagattcaaattcgtggagaaattcattcaaatgttgattacacagttgatctcttgaatgcctcagacttcaaagaaaacaggattcatactggctggctggataacagaatagcaatgcgagtccaagctgagagacctccgtggtatatttcagtggttggaggagctctatataaaacaataacgagcaacacagacactgtttctgaatatgttagctatctcgtcaagggtcagattccaccgaagcatatatcccttgtccattcaactgtttctttgaatatagaggaaagcaaatatacaattgaaactataaggagcggacagggtagctacagattgcgaatgaatggatcagttattgaagcaaatgtccaaacattatgtgatggtggacttttaatgcagttggatggaaacagccatgtaatttatgctgaagaagaggccggtggtacacggcttctaattgatggaaagacatgcttgttacagaatgatcacgatccttcaaggttattagctgagacaccctgcaaacttcttcgtttcttggttgccgatggtgctcatgttgaagctgatgtaccatatgcggaagttgaggttatgaagatgtgcatgcccctcttgtcacctgctgctggtgtcattaatgttttgttgtctgagggccagcctatgcaggctggtgatcttatagcaagacttgatcttgatgacccttctgctgtgaagagagctgagccgtttaacggatctttcccagaaatgagccttcctattgctgcttctggccaagttcacaaaagatgtgccacaagcttgaatgctgctcggatggtccttgcaggatatgatcacccgatcaacaaagttgtacaagatctggtatcctgtctagatgctcctgagcttcctttcctacaatgggaagagcttatgtctgttttagcaactagacttccaaggcttcttaagagcgagttggagggtaaatacagtgaatataagttaaatgttggccatggaaagagcaaggatttcccttccaagatgctaagagagataatcgaggaaaatcttgcacatggttctgagaaggaaattgctacaaatgagaggcttgttgagcctcttatgagcctactgaagtcatatgagggtggcagagaaagccatgcacactttattgtgaagtcccttttcgaggactatctctcggttgaggaactattcagtgatggcattcagtctgatgtgattgaacgcctgcgccaacaacatagtaaagatctccagaaggttgtagacattgtgttgtctcaccagggtgtgagaaacaaaactaagctgatactaacactcatggagaaactggtctatccaaaccctgctgcctacaaggatcagttgactcgcttttcctccctcaatcacaaaagatattataagttggcccttaaagctagcgagcttcttgaacaaaccaagcttagtgagctccgcacaagcattgcaaggagcctttcagaacttgagatgtttactgaagaaaggacggccattagtgagatcatgggagatttagtgactgccccactgccagttgaagatgcactggtttctttgtttgattgtagtgatcaaactcttcagcagagggtgatcgagacgtacatatctcgattataccagcctcatcttgtcaaggatagtatccagctgaaatatcaggaatctggtgttattgctttatgggaattcgctgaagcgcattcagagaagagattgggtgctatggttattgtgaagtcgttagaatctgtatcagcagcaattggagctgcactaaagggtacatcacgctatgcaagctctgagggtaacataatgcatattgctttattgggtgctgataatcaaatgcatggaactgaagacagtggtgataacgatcaagctcaagtcaggatagacaaactttctgcgacactggaacaaaatactgtcacagctgatctccgtgctgctggtgtgaaggttattagttgcattgttcaaagggatggagcactcatgcctatgcgccataccttcctcttgtcggatgaaaagctttgttatgaggaagagccggttctccggcatgtggagcctcctctttctgctcttcttgagttgggtaagttgaaagtgaaaggatacaatgaggtgaagtatacaccgtcacgtgatcgtcagtggaacatatacacacttagaaatacagagaaccccaaaatgttgcacagggtgtttttccgaactcttgtcaggcaacccggtgcttccaacaaattcacatcaggcaacatcagtgatgttgaagtgggaggagctgaggaatctctttcatttacatcgagcagcatattaagatcgctgatgactgctatagaagagttggagcttcacgcgattaggacaggtcactctcatatgtttttgtgcatattgaaagagcaaaagcttcttgatcttgttcccgtttcagggaacaaagttgtggatattggccaagatgaagctactgcatgcttgcttctgaaagaaatggctctacagatacatgaacttgtgggtgcaaggatgcatcatctttctgtatgccaatgggaggtgaaacttaagttggacagcgatgggcctgccagtggtacctggagagttgtaacaaccaatgttactagtcacacctgcactgtggatatctaccgtgaggttgaagatacagaatcacagaaactagtgtaccactctgctccatcgtcatctggtcctttgcatggcgttgcactgaatactccatatcagcctttgagtgttattgatctgaaacgttgctccgctagaaataacagaactacatactgctatgattttccgttggcatttgaaactgcagtgcagaagtcatggtctaacatttctagtgacactaaccgatgttatgttaaagcgacggagctggtgtttgctcacaagaacgggtcatggggcactcctgtaattcctatggagcgtcctgctgggctcaatgacattggtatggtagcttggatcttggacatgtccactcctgaatatcccaatggcaggcagattgttgtcatcgcaaatgatattacttttagagctggatcgtttggtccaagggaagatgcattttttgaaactgttaccaacctagcttgtgagaggaagcttcctctcatctacttggcagcaaactctggtgctcggatcggcatagcagatgaagtaaaatcttgcttccgtgttggatggtctgatgatggcagccctgaacgtgggtttcaatatatttatctgactgaagaagaccatgctcgtattagcgcttctgttatagcgcacaagatgcagcttgataatggtgaaattaggtgggttattgattctgttgtagggaaggaggatgggctaggtgtggagaacatacatggaagtgctgctattgccagtgcctattctagggcctatgaggagacatttacgcttacatttgtgactggaaggactgttggaataggagcatatcttgctcgacttggcatacggtgcattcagcgtactgaccagcccattatcctaactgggttctctgccttgaacaagcttcttggccgggaagtgtacagctcccacatgcagttgggtggccccaaaattatggccacaaacggtgttgtccatctgacagtttcagatgaccttgaaggtgtatctaatatattgaggtggctcagctatgttcctgccaacattggtggacctcttcctattacaaaatctttggacccacctgacagacccgttgcttacatccctgagaatacatgtgatcctcgtgcagccatcagtggcattgatgatagccaagggaaatggttggggggtatgttcgacaaagacagttttgtggagacatttgaaggatgggcgaagtcagtagttactggcagagcgaaactcggagggattccggtgggtgttatagctgtggagacacagactatgatgcagctcatccctgctgatccaggtcagcttgattcccatgagcggtctgttcctcgtgctgggcaagtctggtttccagattcagctactaagacagcgcaggcaatgctggacttcaaccgtgaaggattacctctgttcatccttgctaactggagaggcttctctggtgggcaaagagatctttttgaaggaatccttcaggctgggtcaacaattgttgagaaccttaggacatacaatcagcctgcctttgtatatatccccaaggctgcagagctacgtggaggggcttgggtcgtgattgatagcaagataaatccagatcgcattgagttctatgctgagaggactgcaaagggcaatgttcttgaacctcaagggttgattgagatcaagttcaggtcagaggaactccaagagtgcatgggcaggcttgacccagaattgataaatttgaaggcaaaactcctgggagcaaagcatgaaaatggaagtctatctgagtcagaatcccttcagaagagcatagaagcccggaagaaacagttgttgcctttgtatactcaaattgcggtacggttcgctgaattgcatgacacttcccttagaatggctgctaagggtgtgattaagaaggttgtagactgggaagattctaggtctttcttctacaagagattacggaggaggatatccgaggatgttcttgcaaaggaaattagaggtgtaagtggcaagcagttttctcaccaatcggcaatcgagctgatccagaaatggtacttggcctctaagggagctgaaacgggaaacactgaatgggatgatgacgatgcttttgttgcctggagggaaaaccctgaaaactaccaggagtatatcaaagaactcagggctcaaagggtatctcagttgctctcagatgttgcagactccagtccagatctagaagccttgccacagggtctttctatgctactagagaagatggatccctcaaggagagcacagtttgttgaggaagtcaagaaggcccttaaatga

SEQ ID NO: 26 - protein, 2311 aa, Aegilops tauschii
MGSTHLPIVGLNASTTPSLSTIRPVNSAGAAFQPSAPSRTSKKKSRRVQSLRDGGDGGVSDPNQSIRQGLAGIIDLPKEGTSAPEVDISHGSEEPRGSYQMNGILNEAHNGRHASLSKVVEFCMALGGKTPIHSVLVANNGMAAAKFMRSVRTWANETFGSEKAIQLIAMATPEDMRINAEHIRIADQFVEVPGGTNNNNYANVQLIVEIAVRTGVSAVWPGWGHASENPELPDALNANGIVFLGPPSSSMNALGDKVGSALIAQAAGVPTLPWSGSQVEIPLEVCLDSIPADMYRKACVSTTEEALASCQMIGYPAMIKASWGGGGKGIRKVNNDDDVRALFKQVQGEVPGSPIFIMRLASQSRHLEVQLLCDQYGNVAALHSRDCSVQRRHQKIIEEGPVTVAPRETVKELEQAARRLAKAVGYVGAATVEYLYSMETGEYYFLELNPRLQVEHPVTEWIAEVNLPAAQVAVGMGIPLWQVPEIRRFYGMDNGGGYDIWRKTAALATPFNFDEVDSQWPKGHCVAVRITSEDPDDGFKPTGGKVKEISFKSKPNVWAYFSVKSGGGIHEFADSQFGHVFAYGVSRAAAITNMSLALKEIQIRGEIHSNVDYTVDLLNASDFKENRIHTGWLDNRIAMRVQAERPPWYISVVGGALYKTITSNTDTVSEYVSYLVKGQIPPKHISLVHSTVSLNIEESKYTIETIRSGQGSYRLRMNGSVIEANVQTLCDGGLLMQLDGNSHVIYAEEEAGGTRLLIDGKTCLLQNDHDPSRLLAETPCKLLRFLVADGAHVEADVPYAEVEVMKMCMPLLSPAAGVINVLLSEGQPMQAGDLIARLDLDDPSAVKRAEPFNGSFPEMSLPIAASGQVHKRCATSLNAARMVLAGYDHPINKVVQDLVSCLDAPELPFLQWEELMSVLATRLPRLLKSELEGKYSEYKLNVGHGKSKDFPSKMLREIIEENLAHGSEKEIATNERLVEPLMSLLKSYEGGRESHAHFIVKSLFEDYLSVEELFSDGIQSDVIERLRQQHSKDLQKVVDIVLSHQGVRNKTKLILTLMEKLVYPNPAAYKDQLTRFSSLNHKRYYKLALKASELLEQTKLSELRTSIARSLSELEMFTEERTAISEIMGDLVTAPLPVEDALVSLFDCSDQTLQQRVIETYISRLYQPHLVKDSIQLKYQESGVIALWEFAEAHSEKRLGAMVIVKSLESVSAAIGAALKGTSRYASSEGNIMHIALLGADNQMHGTEDSGDNDQAQVRIDKLSATLEQNTVTADLRAAGVKVISCIVQRDGALMPMRHTFLLSDEKLCYEEEPVLRHVEPPLSALLELGKLKVKGYNEVKYTPSRDRQWNIYTLRNTENPKMLHRVFFRTLVRQPGASNKFTSGNISDVEVGGAEESLSFTSSSILRSLMTAIEELELHAIRTGHSHMFLCILKEQKLLDLVPVSGNKVVDIGQDEATACLLLKEMALQIHELVGARMHHLSVCQWEVKLKLDSDGPASGTWRVVTTNVTSHTCTVDIYREVEDTESQKLVYHSAPSSSGPLHGVALNTPYQPLSVIDLKRCSARNNRTTYCYDFPLAFETAVQKSWSNISSDTNRCYVKATELVFAHKNGSWGTPVIPMERPAGLNDIGMVAWILDMSTPEYPNGRQIVVIANDITFRAGSFGPREDAFFETVTNLACERKLPLIYLAANSGARIGIADEVKSCFRVGWSDDGSPERGFQYIYLTEEDHARISASVIAHKMQLDNGEIRWVIDSVVGKEDGLGVENIHGSAAIASAYSRAYEETFTLTFVTGRTVGIGAYLARLGIRCIQRTDQPIILTGFSALNKLLGREVYSSHMQLGGPKIMATNGVVHLTVSDDLEGVSNILRWLSYVPANIGGPLPITKSLDPPDRPVAYIPENTCDPRAAISGIDDSQGKWLGGMFDKDSFVETFEGWAKSVVTGRAKLGGIPVGVIAVETQTMMQLIPADPGQLDSHERSVPRAGQVWFPDSATKTAQAMLDFNREGLPLFILANWRGFSGGQRDLFEGILQAGSTIVENLRTYNQPAFVYIPKAAELRGGAWVVIDSKINPDRIEFYAERTAKGNVLEPQGLIEIKFRSEELQECMGRLDPELINLKAKLLGAKHENGSLSESESLQKSIEARKKQLLPLYTQIAVRFAELHDTSLRMAAKGVIKKVVDWEDSRSFFYKRLRRRISEDVLAKEIRGVSGKQFSHQSAIELIQKWYLASKGAETGNTEWDDDDAFVAWRENPENYQEYIKELRAQRVSQLLSDVADSSPDLEALPQGLSMLLEKMDPSRRAQFVEEVKKALK